European Patent Application EP 4 745 159 A1, published May 20, 2026. Title: 细胞免疫疗法的组合物和方法. Applicant: 科济生物医药（上海）有限公司. The sequence listing filed with the application follows.

SEQUENCE LISTING (117 sequences)

SEQ ID NO: 1 - protein, 21 aa, synthetic construct
MALPVTALLLPLALLLHAARP

SEQ ID NO: 2 - protein, 22 aa, synthetic construct
MLLLVTSLLLCELPHPAFLLIP

SEQ ID NO: 3 - protein, 45 aa, synthetic construct
TTTPAPRPPTPAPTIASQPLSLRPEACRPAAGGAVHTRGLDFACD

SEQ ID NO: 4 - DNA, 2928 bp, synthetic construct
  source 1..2928: mol_type = other DNA
atggccttaccagtgaccgccttgctcctgccgctggccttgctgctccacgccgccaggccgcaggtgcagctggtgcagagcggcgccgaggtgaagaagcccggcgccagcgtgaaggtgagctgcaaggccagcggctacaccttcaccagctactggatgaactgggtgcggcaggcccccggccagggcctggagtggatgggccggatcgacccctacgacagcgagacccactacgcccagaagctgcagggccgggtgaccatgaccaccgacaccagcaccagcaccgcctacatggagctgcggagcctgcggagcgacgacaccgccgtgtactactgcgcccggggcggctacgacttcgacgtgggcaccctgtactggttcttcgacgtgtggggccagggcaccaccgtgaccgtgagcagcggtggaggcggttcaggcggaggtggttctggcggtggcggatcggacatccagatgacccagagccccagcagcctgagcgccagcgtgggcgaccgggtgaccatcacctgccgggccagcgagaacatctacagctacctggcctggtaccagcagaagcccggcaaggcccccaagctgctgatctacaacgccaagaccctggccgagggcgtgcccagccggttcagcggcagcggcagcggcaccgacttcaccctgaccatcagcagcctgcagcccgaggacttcgccacctactactgccagcaccactacggcaccccccggaccttcggcggcggcaccaaggtggagatcaagaccacgacgccagcgccgcgaccaccaacaccggcgcccaccatcgcgtcgcagcccctgtccctgcgcccagaggcgtgccggccagcggcggggggcgcagtgcacacgagggggctggacttcgcctgtgatttttgggtgctggtggtggttggtggagtcctggcttgctatagcttgctagtaacagtggcctttattattttctgggtgaggagtaagaggagcaggctcctgcacagtgactacatgaacatgactccccgccgccccgggccaacccgcaagcattaccagccctatgccccaccacgcgacttcgcagcctatcgctccagagtgaagttcagcaggagcgcagacgcccccgcgtaccagcagggccagaaccagctctataacgagctcaatctaggacgaagagaggagtacgatgttttggacaagagacgtggccgggaccctgagatggggggaaagccgcagagaaggaagaaccctcaggaaggcctgtacaatgaactgcagaaagataagatggcggaggcctacagtgagattgggatgaaaggcgagcgccggaggggcaaggggcacgatggcctttaccagggtctcagtacagccaccaaggacacctacgacgcccttcacatgcaggccctgccccctcgcggaagcggagctactaacttcagcctgctgaagcaggctggagacgtggaggagaaccctgggcccatggctctgcctgtgacagctctgctgctgcctctggctctgcttctgcatgccgctagacctgaagtgcagctgctggaatctggcggaggactggttcaacctggcggctctctgagactgagctgtgccgtgtccggcttcaccttcaacagcttcgccatgagctgggtccgacaggcccctggaaaaggccttgaatgggtgtccgccatctctggaagcggcggaggcacatattacgccgactctgtgaagggcagattcaccatcagccgggacaacagcaagaacaccctgtacctgcagatgaactccctgagagccgaggataccgccgtgtacttctgcgccaaggacaagatcctttggttcggcgagcccgtgttcgactattggggacagggaaccctggtcaccgtttctagcggaggcggaggttctggtggtggtggatcaggtggcggcggatctgagattgtgctgacacagtctcccgccacactgtctcttagccctggcgaaagagccacactgagctgcagagccagccagagcgtgtcctcttacctggcctggtatcagcagaagcccggccaagctcctcggctgctgatctacgatgccagcaatagagccacaggcatccctgccagattttccggctctggcagcggcaccgatttcaccctgaccataagcagcctggaacctgaggacttcgccgtgtattactgccagcagcggagcaactggcctcctacatttggccagggaaccaaagtcgagatcaaggagtctaagtacggccctccttgtcctccatgtcctatgttttgggtcctcgtcgtcgtcggaggcgtgctggcttgctatagcctgcttgtgacagtggcctttattatcttctgggttagaagcaagcggagccggctgctgcacagcgactacatgaacatgacccctagacggcccggacctaccagaaagcactaccagccttacgctcctcctcgggatttcgccgcctacagatctcgcgtgaaattctccagaagcgctgacgcccctgcttatcagcaaggccagaatcagctctataacgaactcaatctcggcaggcgcgaggaatatgatgtgctggataagaggcgcggcagggacccagaaatgggaggaaaacctcagcggcggaaaaacccacaagaaggcctttacaacgaactgcaaaaggataagatggcagaagcttactccgagattggcatgaagggcgaacgtcggagaggaaaaggccacgacggactctatcagggactgtctacagccacaaaggacacatacgacgcactccatatgcaggctctcccacctagatag

SEQ ID NO: 5 - protein, 228 aa, synthetic construct
ESKYGPPCPPCPAPPVAGPSVFLFPPKPKDTLMISRTPEVTCVVVDVSQEDPEVQFNWYVDGVEVHNAKTKPREEQFQSTYRVVSVLTVLHQDWLNGKEYKCKVSNKGLPSSIEKTISKAKGQPREPQVYTLPPSQEEMTKNQVSLTCLVKGFYPSDIAVEWESNGQPENNYKTTPPVLDSDGSFFLYSRLTVDKSRWQEGNVFSCSVMHEALHNHYTQKSLSLSLGK

SEQ ID NO: 6 - protein, 12 aa, synthetic construct
ESKYGPPCPPCP

SEQ ID NO: 7 - protein, 24 aa, synthetic construct
IYIWAPLAGTCGVLLLSLVITLYC

SEQ ID NO: 8 - protein, 27 aa, synthetic construct
FWVLVVVGGVLACYSLLVTVAFIIFWV

SEQ ID NO: 9 - protein, 28 aa, synthetic construct
MFWVLVVVGGVLACYSLLVTVAFIIFWV

SEQ ID NO: 10 - protein, 41 aa, synthetic construct
RSKRSRLLHSDYMNMTPRRPGPTRKHYQPYAPPRDFAAYRS

SEQ ID NO: 11 - protein, 42 aa, synthetic construct
KRGRKKLLYIFKQPFMRPVQTTQEEDGCSCRFPEEEEGGCEL

SEQ ID NO: 12 - protein, 113 aa, synthetic construct
RVKFSRSADAPAYQQGQNQLYNELNLGRREEYDVLDKRRGRDPEMGGKPQRRKNPQEGLYNELQKDKMAEAYSEIGMKGERRRGKGHDGLYQGLSTATKDTYDALHMQALPPR

SEQ ID NO: 13 - protein, 112 aa, synthetic construct
RVKFSRSADAPAYQQGQNQLYNELNLGRREEYDVLDKRRGRDPEMGGKPRRKNPQEGLYNELQKDKMAEAYSEIGMKGERRRGKGHDGLYQGLSTATKDTYDALHMQALPPR

SEQ ID NO: 14 - protein, 15 aa, synthetic construct
GGGGSGGGGSGGGGS

SEQ ID NO: 15 - protein, 18 aa, synthetic construct
GSTSGSGKPGSGEGSTKG

SEQ ID NO: 16 - DNA, 45 bp, synthetic construct
  source 1..45: mol_type = other DNA
ggcggaggtggaagcggaggcggaggatcgggcggcggaggaagc

SEQ ID NO: 17 - DNA, 57 bp, synthetic construct
  source 1..57: mol_type = other DNA
gctactaacttcagcctgctgaagcaggctggagacgtggaggagaaccctgggccc

SEQ ID NO: 18 - DNA, 1380 bp, synthetic construct
  source 1..1380: mol_type = other DNA
atggctctgcctgtgacagctctgctgctgcctctggctctgcttctgcatgccgctagacctcaggtgcagctggtggagagcggcggcggcctggtgcagcccggcggcagcctgcggctgagctgcgccgccagcggcttcaccttcagcagctactacatgaactgggtgcggcaggcccccggcaagggcctggagtgggtgagcggcatcagcggcgaccccagcaacacctactacgccgacagcgtgaagggccggttcaccatcagccgggacaacagcaagaacaccctgtacctgcagatgaacagcctgcgggccgaggacaccgccgtgtactactgcgcccgggacctgcccctggtgtacaccggcttcgcctactggggccagggcaccctggtgaccgtgagcagcggtggaggcggttcaggcggaggtggttctggcggtggcggatcggacatcgagctgacccagccccccagcgtgagcgtggcccccggccagaccgcccggatcagctgcagcggcgacaacctgcggcactactacgtgtactggtaccagcagaagcccggccaggcccccgtgctggtgatctacggcgacagcaagcggcccagcggcatccccgagcggttcagcggcagcaacagcggcaacaccgccaccctgaccatcagcggcacccaggccgaggacgaggccgactactactgccagacctacaccggcggcgccagcctggtgttcggcggcggcaccaagctgaccgtgctgggccaggagtctaagtacggccctccttgtcctccatgtcctatgttctgggtgctcgtggttgttggcggagtgctggcctgttactctctgctggtgaccgtggccttcatcatcttttgggtcaagcggggcagaaagaagctgctgtacatcttcaagcagcccttcatgcggcccgtgcagaccacacaagaggaagatggctgctcctgcagattccccgaggaagaagaaggcggctgcgagctgagagtgaagttcagcagatccgccgacgctcctgcctatcagcagggacagaaccagctgtacaacgagctgaacctcgggagaagagaagagtacgacgtgctggacaagcggagaggcagagatcctgagatgggcggaaagccccagcggagaaagaatcctcaagagggcctgtataatgagctgcagaaagacaagatggccgaggcctacagcgagatcggaatgaagggcgagcgcagaagaggcaagggacacgatggactgtaccagggcctgagcaccgccaccaaggatacctatgatgccctgcacatgcaggccctgcctccaaga

SEQ ID NO: 19 - protein, 244 aa, synthetic construct
EVQLLESGGGLVQPGGSLRLSCAVSGFTFNSFAMSWVRQAPGKGLEWVSAISGSGGGTYYADSVKGRFTISRDNSKNTLYLQMNSLRAEDTAVYFCAKDKILWFGEPVFDYWGQGTLVTVSSGGGGSGGGGSGGGGSEIVLTQSPATLSLSPGERATLSCRASQSVSSYLAWYQQKPGQAPRLLIYDASNRATGIPARFSGSGSGTDFTLTISSLEPEDFAVYYCQQRSNWPPTFGQGTKVEIK

SEQ ID NO: 20 - protein, 244 aa, synthetic construct
QVQLVESGGGLVQPGGSLRLSCAASGFTFSSYYMNWVRQAPGKGLEWVSGISGDPSNTYYADSVKGRFTISRDNSKNTLYLQMNSLRAEDTAVYYCARDLPLVYTGFAYWGQGTLVTVSSGGGGSGGGGSGGGGSDIELTQPPSVSVAPGQTARISCSGDNLRHYYVYWYQQKPGQAPVLVIYGDSKRPSGIPERFSGSNSGNTATLTISGTQAEDEADYYCQTYTGGASLVFGGGTKLTVLGQ

SEQ ID NO: 21 - protein, 242 aa, synthetic construct
QVQLVQSGAEVAKPGTSVKLSCKASGYTFTDYWMQWVKQRPGQGLEWIGTIYPGDGDTGYAQKFQGKATLTADKSSKTVYMHLSSLASEDSAVYYCARGDYYGSNSLDYWGQGTSVTVSSGGGGSGGGGSGGGGSDIVMTQSHLSMSTSLGDPVSITCKASQDVSTVVAWYQQKPGQSPRRLIYSASYRYIGVPDRFTGSGAGTDFTFTISSVQAEDLAVYYCQQHYSPPYTFGGGTKLEIK

SEQ ID NO: 22 - protein, 243 aa, synthetic construct
QVQLVQSGAEVKKPGSSVKVSCKAFGGTFSSYAISWVRQAPGQGLEWMGRIIRFLGIANYAQKFQGRVTLIADKSTNTAYMELSSLRSEDTAVYYCAGEPGERDPDAVDIWGQGTMVTVSSGGGGSGGGGSGGGGSDIQMTQSPSSLSASVGDRVTITCRASQGISNYLAWFQQKPGKAPKSLIYAASSLQSGVPSRFSGSGSGTDFTLTISSLQPEDFATYYCQQYNSYPYTFGQGTKLEIK

SEQ ID NO: 23 - DNA, 1380 bp, synthetic construct
  source 1..1380: mol_type = other DNA
atggccttaccagtgaccgccttgctcctgccgctggccttgctgctccacgccgccaggccggaggtgcagctgctggagagcggcggcggcctggtgcagcccggcggcagcctgcggctgagctgcgccgtgagcggcttcaccttcaacagcttcgccatgagctgggtgcggcaggcccccggcaagggcctggagtgggtgagcgccatcagcggcagcggcggcggcacctactacgccgacagcgtgaagggccggttcaccatcagccgggacaacagcaagaacaccctgtacctgcagatgaacagcctgcgggccgaggacaccgccgtgtacttctgcgccaaggacaagatcctgtggttcggcgagcccgtgttcgactactggggccagggcaccctggtgaccgtgagcagcggtggaggcggttcaggcggaggtggttctggcggtggcggatcggagatcgtgctgacccagagccccgccaccctgagcctgagccccggcgagcgggccaccctgagctgccgggccagccagagcgtgagcagctacctggcctggtaccagcagaagcccggccaggccccccggctgctgatctacgacgccagcaaccgggccaccggcatccccgcccggttcagcggcagcggcagcggcaccgacttcaccctgaccatcagcagcctggagcccgaggacttcgccgtgtactactgccagcagcggagcaactggccccccaccttcggccagggcaccaaggtggagatcaaggagtccaaatatggtcccccatgcccaccatgcccaatgttttgggtgctggtggtggttggtggagtcctggcttgctatagcttgctagtaacagtggcctttattattttctgggtgaaacggggcagaaagaaactcctgtatatattcaaacaaccatttatgagaccagtacaaactactcaagaggaagatggctgtagctgccgatttccagaagaagaagaaggaggatgtgaactgagagtgaagttcagcaggagcgcagacgcccccgcgtaccagcagggccagaaccagctctataacgagctcaatctaggacgaagagaggagtacgatgttttggacaagagacgtggccgggaccctgagatggggggaaagccgcagagaaggaagaaccctcaggaaggcctgtacaatgaactgcagaaagataagatggcggaggcctacagtgagattgggatgaaaggcgagcgccggaggggcaaggggcacgatggcctttaccagggtctcagtacagccaccaaggacacctacgacgcccttcacatgcaggccctgccccctcgc

SEQ ID NO: 24 - protein, 460 aa, synthetic construct
MALPVTALLLPLALLLHAARPEVQLLESGGGLVQPGGSLRLSCAVSGFTFNSFAMSWVRQAPGKGLEWVSAISGSGGGTYYADSVKGRFTISRDNSKNTLYLQMNSLRAEDTAVYFCAKDKILWFGEPVFDYWGQGTLVTVSSGGGGSGGGGSGGGGSEIVLTQSPATLSLSPGERATLSCRASQSVSSYLAWYQQKPGQAPRLLIYDASNRATGIPARFSGSGSGTDFTLTISSLEPEDFAVYYCQQRSNWPPTFGQGTKVEIKESKYGPPCPPCPMFWVLVVVGGVLACYSLLVTVAFIIFWVKRGRKKLLYIFKQPFMRPVQTTQEEDGCSCRFPEEEEGGCELRVKFSRSADAPAYQQGQNQLYNELNLGRREEYDVLDKRRGRDPEMGGKPQRRKNPQEGLYNELQKDKMAEAYSEIGMKGERRRGKGHDGLYQGLSTATKDTYDALHMQALPPR

SEQ ID NO: 25 - DNA, 1377 bp, synthetic construct
  source 1..1377: mol_type = other DNA
atggctctgcctgtgacagctctgctgctgcctctggctctgcttctgcatgccgctagacctgaagtgcagctgctggaatctggcggaggactggttcaacctggcggctctctgagactgagctgtgccgtgtccggcttcaccttcaacagcttcgccatgagctgggtccgacaggcccctggaaaaggccttgaatgggtgtccgccatctctggaagcggcggaggcacatattacgccgactctgtgaagggcagattcaccatcagccgggacaacagcaagaacaccctgtacctgcagatgaactccctgagagccgaggataccgccgtgtacttctgcgccaaggacaagatcctttggttcggcgagcccgtgttcgactattggggacagggaaccctggtcaccgtttctagcggaggcggaggttctggtggtggtggatcaggtggcggcggatctgagattgtgctgacacagtctcccgccacactgtctcttagccctggcgaaagagccacactgagctgcagagccagccagagcgtgtcctcttacctggcctggtatcagcagaagcccggccaagctcctcggctgctgatctacgatgccagcaatagagccacaggcatccctgccagattttccggctctggcagcggcaccgatttcaccctgaccataagcagcctggaacctgaggacttcgccgtgtattactgccagcagcggagcaactggcctcctacatttggccagggaaccaaagtcgagatcaaggagtctaagtacggccctccttgtcctccatgtcctatgttttgggtcctcgtcgtcgtcggaggcgtgctggcttgctatagcctgcttgtgacagtggcctttattatcttctgggttagaagcaagcggagccggctgctgcacagcgactacatgaacatgacccctagacggcccggacctaccagaaagcactaccagccttacgctcctcctcgggatttcgccgcctacagatctcgcgtgaaattctccagaagcgctgacgcccctgcttatcagcaaggccagaatcagctctataacgaactcaatctcggcaggcgcgaggaatatgatgtgctggataagaggcgcggcagggacccagaaatgggaggaaaacctcagcggcggaaaaacccacaagaaggcctttacaacgaactgcaaaaggataagatggcagaagcttactccgagattggcatgaagggcgaacgtcggagaggaaaaggccacgacggactctatcagggactgtctacagccacaaaggacacatacgacgcactccatatgcaggctctcccacctaga

SEQ ID NO: 26 - protein, 459 aa, synthetic construct
MALPVTALLLPLALLLHAARPEVQLLESGGGLVQPGGSLRLSCAVSGFTFNSFAMSWVRQAPGKGLEWVSAISGSGGGTYYADSVKGRFTISRDNSKNTLYLQMNSLRAEDTAVYFCAKDKILWFGEPVFDYWGQGTLVTVSSGGGGSGGGGSGGGGSEIVLTQSPATLSLSPGERATLSCRASQSVSSYLAWYQQKPGQAPRLLIYDASNRATGIPARFSGSGSGTDFTLTISSLEPEDFAVYYCQQRSNWPPTFGQGTKVEIKESKYGPPCPPCPMFWVLVVVGGVLACYSLLVTVAFIIFWVRSKRSRLLHSDYMNMTPRRPGPTRKHYQPYAPPRDFAAYRSRVKFSRSADAPAYQQGQNQLYNELNLGRREEYDVLDKRRGRDPEMGGKPQRRKNPQEGLYNELQKDKMAEAYSEIGMKGERRRGKGHDGLYQGLSTATKDTYDALHMQALPPR

SEQ ID NO: 27 - protein, 460 aa, synthetic construct
MALPVTALLLPLALLLHAARPQVQLVESGGGLVQPGGSLRLSCAASGFTFSSYYMNWVRQAPGKGLEWVSGISGDPSNTYYADSVKGRFTISRDNSKNTLYLQMNSLRAEDTAVYYCARDLPLVYTGFAYWGQGTLVTVSSGGGGSGGGGSGGGGSDIELTQPPSVSVAPGQTARISCSGDNLRHYYVYWYQQKPGQAPVLVIYGDSKRPSGIPERFSGSNSGNTATLTISGTQAEDEADYYCQTYTGGASLVFGGGTKLTVLGQESKYGPPCPPCPMFWVLVVVGGVLACYSLLVTVAFIIFWVKRGRKKLLYIFKQPFMRPVQTTQEEDGCSCRFPEEEEGGCELRVKFSRSADAPAYQQGQNQLYNELNLGRREEYDVLDKRRGRDPEMGGKPQRRKNPQEGLYNELQKDKMAEAYSEIGMKGERRRGKGHDGLYQGLSTATKDTYDALHMQALPPR

SEQ ID NO: 28 - protein, 458 aa, synthetic construct
MALPVTALLLPLALLLHAARPQVQLVQSGAEVAKPGTSVKLSCKASGYTFTDYWMQWVKQRPGQGLEWIGTIYPGDGDTGYAQKFQGKATLTADKSSKTVYMHLSSLASEDSAVYYCARGDYYGSNSLDYWGQGTSVTVSSGGGGSGGGGSGGGGSDIVMTQSHLSMSTSLGDPVSITCKASQDVSTVVAWYQQKPGQSPRRLIYSASYRYIGVPDRFTGSGAGTDFTFTISSVQAEDLAVYYCQQHYSPPYTFGGGTKLEIKESKYGPPCPPCPMFWVLVVVGGVLACYSLLVTVAFIIFWVKRGRKKLLYIFKQPFMRPVQTTQEEDGCSCRFPEEEEGGCELRVKFSRSADAPAYQQGQNQLYNELNLGRREEYDVLDKRRGRDPEMGGKPQRRKNPQEGLYNELQKDKMAEAYSEIGMKGERRRGKGHDGLYQGLSTATKDTYDALHMQALPPR

SEQ ID NO: 29 - DNA, 1374 bp, synthetic construct
  source 1..1374: mol_type = other DNA
atggccttaccagtgaccgccttgctcctgccgctggccttgctgctccacgccgccaggccgcaggtgcagctggtgcagagcggcgccgaggtggccaagcccggcaccagcgtgaagctgagctgcaaggccagcggctacaccttcaccgactactggatgcagtgggtgaagcagcggcccggccagggcctggagtggatcggcaccatctaccccggcgacggcgacaccggctacgcccagaagttccagggcaaggccaccctgaccgccgacaagagcagcaagaccgtgtacatgcacctgagcagcctggccagcgaggacagcgccgtgtactactgcgcccggggcgactactacggcagcaacagcctggactactggggccagggcaccagcgtgaccgtgagcagcggtggaggcggttcaggcggaggtggttctggcggtggcggatcggacatcgtgatgacccagagccacctgagcatgagcaccagcctgggcgaccccgtgagcatcacctgcaaggccagccaggacgtgagcaccgtggtggcctggtaccagcagaagcccggccagagcccccggcggctgatctacagcgccagctaccggtacatcggcgtgcccgaccggttcaccggcagcggcgccggcaccgacttcaccttcaccatcagcagcgtgcaggccgaggacctggccgtgtactactgccagcagcactacagccccccctacaccttcggcggcggcaccaagctggagatcaaggagtccaaatatggtcccccatgcccaccatgcccaatgttttgggtgctggtggtggttggtggagtcctggcttgctatagcttgctagtaacagtggcctttattattttctgggtgaaacggggcagaaagaaactcctgtatatattcaaacaaccatttatgagaccagtacaaactactcaagaggaagatggctgtagctgccgatttccagaagaagaagaaggaggatgtgaactgagagtgaagttcagcaggagcgcagacgcccccgcgtaccagcagggccagaaccagctctataacgagctcaatctaggacgaagagaggagtacgatgttttggacaagagacgtggccgggaccctgagatggggggaaagccgcagagaaggaagaaccctcaggaaggcctgtacaatgaactgcagaaagataagatggcggaggcctacagtgagattgggatgaaaggcgagcgccggaggggcaaggggcacgatggcctttaccagggtctcagtacagccaccaaggacacctacgacgcccttcacatgcaggccctgccccctcgc

SEQ ID NO: 30 - DNA, 1500 bp, synthetic construct
  source 1..1500: mol_type = other DNA
atgtctcgctccgtggctctggccgtcttggccttgttatctctttctggcctggaggctgtcatggcgccccgaaccgtcctcctgggtggtggcggaagcggtggtggcggttctggtggtggcggctccatccagcgtactccaaagattcaggtttactcacgtcatccagcagagaatggaaagtcaaatttcctgaattgctatgtgtctgggtttcatccatccgacattgaagttgacttactgaagaatggagagagaattgaaaaagtggagcattcagacttgtctttcagcaaggactggtctttctatctcttgtactacactgaattcacccccactgaaaaagatgagtatgcctgccgtgtgaaccatgtgactttgtcacagcccaagatagttaagtgggatcgcgacatgggtggtggcggttctggtggtggcggtagtggcggcggaggaagcggtggtggcggttccggatctcactccttgaagtatttccacacttccgtgtcccggcccggccgcggggagccccgcttcatctctgtgggctacgtggacgacacccagttcgtgcgcttcgacaacgacgccgcgagtccgaggatggtgccgcgggcgccgtggatggagcaggaggggtcagagtattgggaccgggagacacggagcgccagggacaccgcacagattttccgagtgaacctgcggacgctgcgcggctactacaatcagagcgaggccgggtctcacaccctgcagtggatgcatggctgcgagctggggcccgacaggcgcttcctccgcgggtatgaacagttcgcctacgacggcaaggattatctcaccctgaatgaggacctgcgctcctggaccgcggtggacacggcggctcagatctccgagcaaaagtcaaatgatgcctctgaggcggagcaccagagagcctacctggaagacacatgcgtggagtggctccacaaatacctggagaaggggaaggagacgctgcttcacctggagcccccaaagacacacgtgactcaccaccccatctctgaccatgaggccaccctgaggtgctgggccctgggcttctaccctgcggagatcacactgacctggcagcaggatggggagggccatacccaggacacggagctcgtggagaccaggcctgcaggggatggaaccttccagaagtgggcagctgtggtggtgccttctggagaggagcagagatacacgtgccatgtgcagcatgaggggctacccgagcccgtcaccctgagatggaagccggcttcccagcccaccatccccatcgtgggcatcattgctggcctggttctccttggatctgtggtctctggagctgtggttgctgctgtgatatggaggaagaagagctcaggtggaaaaggagggagctactctaaggctgagtggagcgacagtgcccaggggtctgagtctcacagcttg

SEQ ID NO: 31 - DNA, 1500 bp, synthetic construct
  source 1..1500: mol_type = other DNA
atgtctcgctccgtggctctggccgtcttggccttgttatctctttctggcctggaggctgtcatggcgccccgagccctcctcctgggtggtggcggaagcggtggtggcggttctggtggtggcggctccatccagcgtactccaaagattcaggtttactcacgtcatccagcagagaatggaaagtcaaatttcctgaattgctatgtgtctgggtttcatccatccgacattgaagttgacttactgaagaatggagagagaattgaaaaagtggagcattcagacttgtctttcagcaaggactggtctttctatctcttgtactacactgaattcacccccactgaaaaagatgagtatgcctgccgtgtgaaccatgtgactttgtcacagcccaagatagttaagtgggatcgcgacatgggtggtggcggttctggtggtggcggtagtggcggcggaggaagcggtggtggcggttccggatctcactccttgaagtatttccacacttccgtgtcccggcccggccgcggggagccccgcttcatctctgtgggctacgtggacgacacccagttcgtgcgcttcgacaacgacgccgcgagtccgaggatggtgccgcgggcgccgtggatggagcaggaggggtcagagtattgggaccgggagacacggagcgccagggacaccgcacagattttccgagtgaacctgcggacgctgcgcggctactacaatcagagcgaggccgggtctcacaccctgcagtggatgcatggctgcgagctggggcccgacaggcgcttcctccgcgggtatgaacagttcgcctacgacggcaaggattatctcaccctgaatgaggacctgcgctcctggaccgcggtggacacggcggctcagatctccgagcaaaagtcaaatgatgcctctgaggcggagcaccagagagcctacctggaagacacatgcgtggagtggctccacaaatacctggagaaggggaaggagacgctgcttcacctggagcccccaaagacacacgtgactcaccaccccatctctgaccatgaggccaccctgaggtgctgggccctgggcttctaccctgcggagatcacactgacctggcagcaggatggggagggccatacccaggacacggagctcgtggagaccaggcctgcaggggatggaaccttccagaagtgggcagctgtggtggtgccttctggagaggagcagagatacacgtgccatgtgcagcatgaggggctacccgagcccgtcaccctgagatggaagccggcttcccagcccaccatccccatcgtgggcatcattgctggcctggttctccttggatctgtggtctctggagctgtggttgctgctgtgatatggaggaagaagagctcaggtggaaaaggagggagctactctaaggctgagtggagcgacagtgcccaggggtctgagtctcacagcttg

SEQ ID NO: 32 - DNA, 1500 bp, synthetic construct
  source 1..1500: mol_type = other DNA
atgtctcgctccgtggctctggccgtcttggccttgttatctctttctggcctggaggctgttatggctccgcggactttaattttaggtggtggcggatccggtggtggcggttctggtggtggcggctccatccagcgtactccaaagattcaggtttactcacgtcatccagcagagaatggaaagtcaaatttcctgaattgctatgtgtctgggtttcatccatccgacattgaagttgacttactgaagaatggagagagaattgaaaaagtggagcattcagacttgtctttcagcaaggactggtctttctatctcttgtactacactgaattcacccccactgaaaaagatgagtatgcctgccgtgtgaaccatgtgactttgtcacagcccaagatagttaagtgggatcgcgacatgggtggtggcggttctggtggtggcggtagtggcggcggaggaagcggtggtggcggttccggatctcactccttgaagtatttccacacttccgtgtcccggcccggccgcggggagccccgcttcatctctgtgggctacgtggacgacacccagttcgtgcgcttcgacaacgacgccgcgagtccgaggatggtgccgcgggcgccgtggatggagcaggaggggtcagagtattgggaccgggagacacggagcgccagggacaccgcacagattttccgagtgaacctgcggacgctgcgcggctactacaatcagagcgaggccgggtctcacaccctgcagtggatgcatggctgcgagctggggcccgacaggcgcttcctccgcgggtatgaacagttcgcctacgacggcaaggattatctcaccctgaatgaggacctgcgctcctggaccgcggtggacacggcggctcagatctccgagcaaaagtcaaatgatgcctctgaggcggagcaccagagagcctacctggaagacacatgcgtggagtggctccacaaatacctggagaaggggaaggagacgctgcttcacctggagcccccaaagacacacgtgactcaccaccccatctctgaccatgaggccaccctgaggtgctgggccctgggcttctaccctgcggagatcacactgacctggcagcaggatggggagggccatacccaggacacggagctcgtggagaccaggcctgcaggggatggaaccttccagaagtgggcagctgtggtggtgccttctggagaggagcagagatacacgtgccatgtgcagcatgaggggctacccgagcccgtcaccctgagatggaagccggcttcccagcccaccatccccatcgtgggcatcattgctggcctggttctccttggatctgtggtctctggagctgtggttgctgctgtgatatggaggaagaagagctcaggtggaaaaggagggagctactctaaggctgagtggagcgacagtgcccaggggtctgagtctcacagcttg

SEQ ID NO: 33 - DNA, 1500 bp, synthetic construct
  source 1..1500: mol_type = other DNA
atgtctcgctccgtggctctggccgtcttggccttgttatctctttctggcctggaggctgttatggctccgcggactttatttttaggtggtggcggatccggtggtggcggttctggtggtggcggctccatccagcgtactccaaagattcaggtttactcacgtcatccagcagagaatggaaagtcaaatttcctgaattgctatgtgtctgggtttcatccatccgacattgaagttgacttactgaagaatggagagagaattgaaaaagtggagcattcagacttgtctttcagcaaggactggtctttctatctcttgtactacactgaattcacccccactgaaaaagatgagtatgcctgccgtgtgaaccatgtgactttgtcacagcccaagatagttaagtgggatcgcgacatgggtggtggcggttctggtggtggcggtagtggcggcggaggaagcggtggtggcggttccggatctcactccttgaagtatttccacacttccgtgtcccggcccggccgcggggagccccgcttcatctctgtgggctacgtggacgacacccagttcgtgcgcttcgacaacgacgccgcgagtccgaggatggtgccgcgggcgccgtggatggagcaggaggggtcagagtattgggaccgggagacacggagcgccagggacaccgcacagattttccgagtgaacctgcggacgctgcgcggctactacaatcagagcgaggccgggtctcacaccctgcagtggatgcatggctgcgagctggggcccgacaggcgcttcctccgcgggtatgaacagttcgcctacgacggcaaggattatctcaccctgaatgaggacctgcgctcctggaccgcggtggacacggcggctcagatctccgagcaaaagtcaaatgatgcctctgaggcggagcaccagagagcctacctggaagacacatgcgtggagtggctccacaaatacctggagaaggggaaggagacgctgcttcacctggagcccccaaagacacacgtgactcaccaccccatctctgaccatgaggccaccctgaggtgctgggccctgggcttctaccctgcggagatcacactgacctggcagcaggatggggagggccatacccaggacacggagctcgtggagaccaggcctgcaggggatggaaccttccagaagtgggcagctgtggtggtgccttctggagaggagcagagatacacgtgccatgtgcagcatgaggggctacccgagcccgtcaccctgagatggaagccggcttcccagcccaccatccccatcgtgggcatcattgctggcctggttctccttggatctgtggtctctggagctgtggttgctgctgtgatatggaggaagaagagctcaggtggaaaaggagggagctactctaaggctgagtggagcgacagtgcccaggggtctgagtctcacagcttg

SEQ ID NO: 34 - DNA, 2928 bp, synthetic construct
  source 1..2928: mol_type = other DNA
atggctctgcctgtgacagctctgctgctgcctctggctctgcttctgcatgccgctagacctgaagtgcagctgctggaatctggcggaggactggttcaacctggcggctctctgagactgagctgtgccgtgtccggcttcaccttcaacagcttcgccatgagctgggtccgacaggcccctggaaaaggccttgaatgggtgtccgccatctctggaagcggcggaggcacatattacgccgactctgtgaagggcagattcaccatcagccgggacaacagcaagaacaccctgtacctgcagatgaactccctgagagccgaggataccgccgtgtacttctgcgccaaggacaagatcctttggttcggcgagcccgtgttcgactattggggacagggaaccctggtcaccgtttctagcggaggcggaggttctggtggtggtggatcaggtggcggcggatctgagattgtgctgacacagtctcccgccacactgtctcttagccctggcgaaagagccacactgagctgcagagccagccagagcgtgtcctcttacctggcctggtatcagcagaagcccggccaagctcctcggctgctgatctacgatgccagcaatagagccacaggcatccctgccagattttccggctctggcagcggcaccgatttcaccctgaccataagcagcctggaacctgaggacttcgccgtgtattactgccagcagcggagcaactggcctcctacatttggccagggaaccaaagtcgagatcaaggagtctaagtacggccctccttgtcctccatgtcctatgttctgggtgctcgtggttgttggcggagtgctggcctgttactctctgctggtgaccgtggccttcatcatcttttgggtcaagcggggcagaaagaagctgctgtacatcttcaagcagcccttcatgcggcccgtgcagaccacacaagaggaagatggctgctcctgcagattccccgaggaagaagaaggcggctgcgagctgagagtgaagttcagcagatccgccgacgctcctgcctatcagcagggacagaaccagctgtacaacgagctgaacctcgggagaagagaagagtacgacgtgctggacaagcggagaggcagagatcctgagatgggcggaaagccccagcggagaaagaatcctcaagagggcctgtataatgagctgcagaaagacaagatggccgaggcctacagcgagatcggaatgaagggcgagcgcagaagaggcaagggacacgatggactgtaccagggcctgagcaccgccaccaaggatacctatgatgccctgcacatgcaggccctgcctccaagaggaagcggagctactaacttcagcctgctgaagcaggctggagacgtggaggagaaccctgggcccatggcactgccagttactgccctgctgctcccacttgcactgctgcttcatgctgccagacctcaggtgcagctggtgcagagcggcgccgaggtgaagaagcccggcgccagcgtgaaggtcagctgcaaggccagcggctacaccttcaccagctactggatgaactgggtgcggcaggcccccggccagggcctggagtggatgggccggatcgacccctacgacagcgagacccactacgcccagaagctgcagggccgggtgaccatgaccaccgacaccagcaccagcaccgcctacatggagctgcggagcctgcggagcgacgacaccgccgtgtactactgcgcccggggcggctacgacttcgacgtgggcaccctgtactggttcttcgacgtgtggggccagggcaccaccgtgaccgtgagcagcggtggaggcggttcaggcggaggtggttctggcggtggcggatcggacatccagatgacccagagccccagcagcctgagcgccagcgtgggcgaccgggtgaccatcacctgccgggccagcgagaacatctacagctacctggcctggtaccagcagaagcccggcaaggcccccaagctgctgatctacaacgccaagaccctggccgagggcgtgcccagccggttcagcggcagcggcagcggcaccgacttcaccctgaccatcagcagcctgcagcccgaggacttcgccacctactactgccagcaccactacggcaccccccggaccttcggcggcggcaccaaggtggagatcaagaccaccacaccagcacctaggccacctactccagctcctaccattgcctctcaacccctgagcctcagacctgaggcatgtagaccagccgcaggcggcgctgttcacacaagaggcctcgactttgcctgtgatttttgggtcctcgtcgtcgtcggaggcgtgctggcttgctatagcctgcttgtgacagtggcctttattatcttctgggttagaagcaagcggagccggctgctgcacagcgactacatgaacatgacccctagacggcccggacctaccagaaagcactaccagccttacgctcctcctcgggatttcgccgcctacagatctcgcgtgaaattctccagaagcgctgacgcccctgcttatcagcaaggccagaatcagctctataacgaactcaatctcggcaggcgcgaggaatatgatgtgctggataagaggcgcggcagggacccagaaatgggaggaaaacctcagcggcggaaaaacccacaagaaggcctttacaacgaactgcaaaaggataagatggcagaagcttactccgagattggcatgaagggcgaacgtcggagaggaaaaggccacgacggactctatcagggactgtctacagccacaaaggacacatacgacgcactccatatgcaggctctcccacctaga

SEQ ID NO: 35 - DNA, 996 bp, synthetic construct
  source 1..996: mol_type = other DNA
atggccttaccagtgaccgccttgctcctgccgctggccttgctgctccacgccgccaggccggaggttcagctgcagcagtctggcgccgaacttgtgaaacctggcgcctctgtgaagctgagctgtaaagccagcggctacaccttcaccagctactggatgcagtgggtcaagcagaggcctggacagggactcgagtggatcggagagatcgaccccagcgacagctacaccaactacaaccagaagttcaagggcaaagccacactgaccgtggacaccagcagcagcacaacctacatgcagctgagcagcctgaccagcgaggatagcgccgtgtactactgtgccagatggggcatggcctacggcaccagctcctactggtacttcgatgtgtggggcaccggcaccaccgtgacagttagttctggcggaggaagcggtggcggatcaggtggtggatctggcggcggatctgacatccagatgacccagacaaccagcagcctgtctgccagcctgggcgatagagtgaccatctcctgtagagccagccaggacatcagcaactacctgaactggtatcagcagaaacccgacggcaccgtgaagctgctgatctactacacctccagactgcacagcggcgtgcccagcagattttctggctctggcagcggcaccgactactccctgacaatcagcaacctggaacaagaggatatcgctacctacttctgccagcaaggcaacaccctgccttggacatttggcggaggcaccaagctggaaatcaagaccaccaccccggcgccgcgcccgccgaccccggcgccgaccattgcgagccagccgctgagcctgcgcccggaagcgtgccgcccggcggcggcggtgcatacccgcggcctggattttgcgtgcgatgcggcggtgctggtgctgctggtgattgtgattattagcctgattgtgctggtggtgatttgg

SEQ ID NO: 36 - DNA, 2919 bp, synthetic construct
  source 1..2919: mol_type = other DNA
atggctctgcctgtgacagctctgctgctgcctctggctctgcttctgcatgccgctagacctgaagtgcagctgctggaatctggcggaggactggttcaacctggcggctctctgagactgagctgtgccgtgtccggcttcaccttcaacagcttcgccatgagctgggtccgacaggcccctggaaaaggccttgaatgggtgtccgccatctctggaagcggcggaggcacatattacgccgactctgtgaagggcagattcaccatcagccgggacaacagcaagaacaccctgtacctgcagatgaactccctgagagccgaggataccgccgtgtacttctgcgccaaggacaagatcctttggttcggcgagcccgtgttcgactattggggacagggaaccctggtcaccgtttctagcggaggcggaggttctggtggtggtggatcaggtggcggcggatctgagattgtgctgacacagtctcccgccacactgtctcttagccctggcgaaagagccacactgagctgcagagccagccagagcgtgtcctcttacctggcctggtatcagcagaagcccggccaagctcctcggctgctgatctacgatgccagcaatagagccacaggcatccctgccagattttccggctctggcagcggcaccgatttcaccctgaccataagcagcctggaacctgaggacttcgccgtgtattactgccagcagcggagcaactggcctcctacatttggccagggaaccaaagtcgagatcaaggagtctaagtacggccctccttgtcctccatgtcctatgttctgggtgctcgtggttgttggcggagtgctggcctgttactctctgctggtgaccgtggccttcatcatcttttgggtcaagcggggcagaaagaagctgctgtacatcttcaagcagcccttcatgcggcccgtgcagaccacacaagaggaagatggctgctcctgcagattccccgaggaagaagaaggcggctgcgagctgagagtgaagttcagcagatccgccgacgctcctgcctatcagcagggacagaaccagctgtacaacgagctgaacctcgggagaagagaagagtacgacgtgctggacaagcggagaggcagagatcctgagatgggcggaaagccccagcggagaaagaatcctcaagagggcctgtataatgagctgcagaaagacaagatggccgaggcctacagcgagatcggaatgaagggcgagcgcagaagaggcaagggacacgatggactgtaccagggcctgagcaccgccaccaaggatacctatgatgccctgcacatgcaggccctgcctccaagaggaagcggagctactaacttcagcctgctgaagcaggctggagacgtggaggagaaccctgggcccatggcactgccagttactgccctgctgctcccacttgcactgctgcttcatgctgccagacctgaggtgcaattgctggagtctgggggaggcttggtacagcctggggggtccatgagactctcctgtgcagcctccggattcacctttagcagttatgccatgagctgggtccgccaggctccagggaaggggctggagtgggtctcagctattagtggtagtggtggtagcacatactacgcagactccgtgaagggccggttcaccatctccagagacaattccaagaacacgctgtatctgcagatgaacagcctgagagccgaggacacggccgtatattactgtgcgaaatacgaaggtcgttacgttctgggtgcaatggactactggggccaaggaaccctggtcaccgtctcgagtggtggaggcggttcaggcggaggtggttctggcggtggcggatcggacatccagatgacccagtctccttccaccctgtctgcatctgtaggagaccgtgtcaccatcacttgccgtgccagtcagagtattagtagctggttggcctggtatcagcagaaaccagggaaagcccctaagctcctgatctatgatgcctccagtttggaaagtggggtcccatcacgtttcagcggcagtggatccgggacagaattcactctcaccatcagcagcttgcagcctgatgattttgcaacttattactgccaacagtacttctcttacccactgacgtttggccagggcaccaaagtcgagatcaagcgtaccaccacaccagcacctaggccacctactccagctcctaccattgcctctcaacccctgagcctcagacctgaggcatgtagaccagccgcaggcggcgctgttcacacaagaggcctcgactttgcctgtgatttttgggtcctcgtcgtcgtcggaggcgtgctggcttgctatagcctgcttgtgacagtggcctttattatcttctgggttagaagcaagcggagccggctgctgcacagcgactacatgaacatgacccctagacggcccggacctaccagaaagcactaccagccttacgctcctcctcgggatttcgccgcctacagatctcgcgtgaaattctccagaagcgctgacgcccctgcttatcagcaaggccagaatcagctctataacgaactcaatctcggcaggcgcgaggaatatgatgtgctggataagaggcgcggcagggacccagaaatgggaggaaaacctcagcggcggaaaaacccacaagaaggcctttacaacgaactgcaaaaggataagatggcagaagcttactccgagattggcatgaagggcgaacgtcggagaggaaaaggccacgacggactctatcagggactgtctacagccacaaaggacacatacgacgcactccatatgcaggctctcccacctaga

SEQ ID NO: 37 - DNA, 3636 bp, synthetic construct
  source 1..3636: mol_type = other DNA
atggcactgccagttactgccctgctgctcccacttgcactgctgcttcatgctgccagacctgaaatcgtgctgacccagtctcctggaactctgtctctgtcccctggcgagagggctaccctgtcttgtagagcctctcagtccgtgtcctccagctatctcgcctggtatcaacaaaagcctgggcaagcccctcggctgctgatatacggggcttcttctcgcgccaccggcattccagacagattcagcggatctggaagcggcacagatttcacactgaccatctctcggctggaacctgaagatttcgctgtctactactgtcagcagtacaagtctcaccccatcacctttggccagggaacaaaggtcgagatcaagagaggtggcggcggtagtcaggtgcagctggtgcagagcggcgccgaggtgaagaagcccggcgccagcgtgaaggtcagctgcaaggccagcggctacaccttcaccagctactggatgaactgggtgcggcaggcccccggccagggcctggagtggatgggccggatcgacccctacgacagcgagacccactacgcccagaagctgcagggccgggtgaccatgaccaccgacaccagcaccagcaccgcctacatggagctgcggagcctgcggagcgacgacaccgccgtgtactactgcgcccggggcggctacgacttcgacgtgggcaccctgtactggttcttcgacgtgtggggccagggcaccaccgtgaccgtgagcagcggtggaggcggttcaggcggaggtggttctggcggtggcggatcggacatccagatgacccagagccccagcagcctgagcgccagcgtgggcgaccgggtgaccatcacctgccgggccagcgagaacatctacagctacctggcctggtaccagcagaagcccggcaaggcccccaagctgctgatctacaacgccaagaccctggccgagggcgtgcccagccggttcagcggcagcggcagcggcaccgacttcaccctgaccatcagcagcctgcagcccgaggacttcgccacctactactgccagcaccactacggcaccccccggaccttcggcggcggcaccaaggtggagatcaagggcggtggtggaagcgaggtccagctgttggaaagtggcggtggtcttgtgcagcctggcggaagcctcagacttagctgtgccgcctccggcttcacattcagcagctacgccatgtcctgggttcgacaagcacccggaaaaggattggagtgggtttcagccatcagcggcagcggaggcagcacttattatgccgatagcgtgaaaggccggttcaccatctccagagacaactccaagaatacgctctatctccagatgaactctctgcgcgccgaagatacagctgtgtactattgcgccagaggctggccctctcctgtgacctttgattactggggacaagggaccctcgtgaccgtttcttctaccaccacaccagcacctaggccacctactccagctcctaccattgcctctcaacccctgagcctcagacctgaggcatgtagaccagccgcaggcggcgctgttcacacaagaggcctcgactttgcctgtgatatctatatttgggctcccctggccgggacctgcggagttcttctgctgtctctcgtgatcacactgtattgcaagagaggccggaagaagctcctctatatctttaaacagccgtttatgcgcccggtccagactacccaagaagaggacggctgtagctgtcggttccctgaagaggaagaaggcggttgcgaactgcgcgtgaaattctccagaagcgctgacgcccctgcttatcagcaaggccagaatcagctctataacgaactcaatctcggcaggcgcgaggaatatgatgtgctggataagaggcgcggcagggacccagaaatgggaggaaaacctcagcggcggaaaaacccacaagaaggcctttacaacgaactgcaaaaggataagatggcagaagcttactccgagattggcatgaagggcgaacgtcggagaggaaaaggccacgacggactctatcagggactgtctacagccacaaaggacacatacgacgcactccatatgcaggctctcccacctagaggaagcggagctactaacttcagcctgctgaagcaggctggagacgtggaggagaaccctgggcccatggctctgcctgtgacagctctgctgctgcctctggctctgcttctgcatgccgctagacctgaagtgcagctgctggaatctggcggaggactggttcaacctggcggctctctgagactgagctgtgccgtgtccggcttcaccttcaacagcttcgccatgagctgggtccgacaggcccctggaaaaggccttgaatgggtgtccgccatctctggaagcggcggaggcacatattacgccgactctgtgaagggcagattcaccatcagccgggacaacagcaagaacaccctgtacctgcagatgaactccctgagagccgaggataccgccgtgtacttctgcgccaaggacaagatcctttggttcggcgagcccgtgttcgactattggggacagggaaccctggtcaccgtttctagcggaggcggaggttctggtggtggtggatcaggtggcggcggatctgagattgtgctgacacagtctcccgccacactgtctcttagccctggcgaaagagccacactgagctgcagagccagccagagcgtgtcctcttacctggcctggtatcagcagaagcccggccaagctcctcggctgctgatctacgatgccagcaatagagccacaggcatccctgccagattttccggctctggcagcggcaccgatttcaccctgaccataagcagcctggaacctgaggacttcgccgtgtattactgccagcagcggagcaactggcctcctacatttggccagggaaccaaagtcgagatcaaggagtctaagtacggccctccttgtcctccatgtcctatgttctgggtgctcgtggttgttggcggagtgctggcctgttactctctgctggtgaccgtggccttcatcatcttttgggtcaagcggggcagaaagaagctgctgtacatcttcaagcagcccttcatgcggcccgtgcagaccacacaagaggaagatggctgctcctgcagattccccgaggaagaagaaggcggctgcgagctgagagtgaagttcagcagatccgccgacgctcctgcctatcagcagggacagaaccagctgtacaacgagctgaacctcgggagaagagaagagtacgacgtgctggacaagcggagaggcagagatcctgagatgggcggaaagccccagcggagaaagaatcctcaagagggcctgtataatgagctgcagaaagacaagatggccgaggcctacagcgagatcggaatgaagggcgagcgcagaagaggcaagggacacgatggactgtaccagggcctgagcaccgccaccaaggatacctatgatgccctgcacatgcaggccctgcctccaaga

SEQ ID NO: 38 - DNA, 3639 bp, synthetic construct
  source 1..3639: mol_type = other DNA
atggcactgccagttactgccctgctgctcccacttgcactgctgcttcatgctgccagacctgaaatcgtgttaacgcagtctccaggcaccctgtctttgtctcctggagaaagagccaccctctcttgccgcgccagtcagagtgttagcagcagctacttagcctggtaccagcagaaacctggccaggctcccaggctcctcatctatggagcatccagcagggccactggcatcccagacaggttcagtggcagtggatccgggacagacttcactctcaccatcagcagactggagcctgaagattttgcagtgtattactgtcagcagtacttcaacccaccagaatacacgttcggccaggggaccaaagtggaaatcaaacgtggtggaggcggttcacaggtgcagctggtgcagagcggcgccgaggtgaagaagcccggcgccagcgtgaaggtcagctgcaaggccagcggctacaccttcaccagctactggatgaactgggtgcggcaggcccccggccagggcctggagtggatgggccggatcgacccctacgacagcgagacccactacgcccagaagctgcagggccgggtgaccatgaccaccgacaccagcaccagcaccgcctacatggagctgcggagcctgcggagcgacgacaccgccgtgtactactgcgcccggggcggctacgacttcgacgtgggcaccctgtactggttcttcgacgtgtggggccagggcaccaccgtgaccgtgagcagcggtggaggcggttcaggcggaggtggttctggcggtggcggatcggacatccagatgacccagagccccagcagcctgagcgccagcgtgggcgaccgggtgaccatcacctgccgggccagcgagaacatctacagctacctggcctggtaccagcagaagcccggcaaggcccccaagctgctgatctacaacgccaagaccctggccgagggcgtgcccagccggttcagcggcagcggcagcggcaccgacttcaccctgaccatcagcagcctgcagcccgaggacttcgccacctactactgccagcaccactacggcaccccccggaccttcggcggcggcaccaaggtggagatcaagggcggtggcggatcggaggtgcaattgctggagtctgggggaggcttggtacagcctggggggtccctgagactctcctgtgcagcctccggattcacctttggcggtaatgccatgtcctgggtccgccaggctccagggaaggggctggagtgggtctcagcaattagtggtaatggtggtagtacattctacgcagactccgtgaagggccggttcaccatctccagagacaattccaagaacacgctgtatctgcagatgaacagcctgagagccgaggacacggccgtatattactgtgcgaaagttcgtccattctggggtactttcgactactggggccaaggaaccctggtcaccgtctcgagtaccaccacaccagcacctaggccacctactccagctcctaccattgcctctcaacccctgagcctcagacctgaggcatgtagaccagccgcaggcggcgctgttcacacaagaggcctcgactttgcctgtgatatctatatttgggctcccctggccgggacctgcggagttcttctgctgtctctcgtgatcacactgtattgcaagagaggccggaagaagctcctctatatctttaaacagccgtttatgcgcccggtccagactacccaagaagaggacggctgtagctgtcggttccctgaagaggaagaaggcggttgcgaactgcgcgtgaaattctccagaagcgctgacgcccctgcttatcagcaaggccagaatcagctctataacgaactcaatctcggcaggcgcgaggaatatgatgtgctggataagaggcgcggcagggacccagaaatgggaggaaaacctcagcggcggaaaaacccacaagaaggcctttacaacgaactgcaaaaggataagatggcagaagcttactccgagattggcatgaagggcgaacgtcggagaggaaaaggtcacgacggactctatcagggactgtctacagccacaaaggacacatacgacgcactccatatgcaggctctcccacctagaggaagcggagctactaacttcagcctgctgaagcaggctggagacgtggaggagaaccctgggcccatggctctgcctgtgacagctctgctgctgcctctggctctgcttctgcatgccgctagacctgaagtgcagctgctggaatctggcggaggactggttcaacctggcggctctctgagactgagctgtgccgtgtccggcttcaccttcaacagcttcgccatgagctgggtccgacaggcccctggaaaaggccttgaatgggtgtccgccatctctggaagcggcggaggcacatattacgccgactctgtgaagggcagattcaccatcagccgggacaacagcaagaacaccctgtacctgcagatgaactccctgagagccgaggataccgccgtgtacttctgcgccaaggacaagatcctttggttcggcgagcccgtgttcgactattggggacagggaaccctggtcaccgtttctagcggaggcggaggttctggtggtggtggatcaggtggcggcggatctgagattgtgctgacacagtctcccgccacactgtctcttagccctggcgaaagagccacactgagctgcagagccagccagagcgtgtcctcttacctggcctggtatcagcagaagcccggccaagctcctcggctgctgatctacgatgccagcaatagagccacaggcatccctgccagattttccggctctggcagcggcaccgatttcaccctgaccataagcagcctggaacctgaggacttcgccgtgtattactgccagcagcggagcaactggcctcctacatttggccagggaaccaaagtcgagatcaaggagtctaagtacggccctccttgtcctccatgtcctatgttctgggtgctcgtggttgttggcggagtgctggcctgttactctctgctggtgaccgtggccttcatcatcttttgggtcaagcggggcagaaagaagctgctgtacatcttcaagcagcccttcatgcggcccgtgcagaccacacaagaggaagatggctgctcctgcagattccccgaggaagaagaaggcggctgcgagctgagagtgaagttcagcagatccgccgacgctcctgcctatcagcagggacagaaccagctgtacaacgagctgaacctcgggagaagagaagagtacgacgtgctggacaagcggagaggcagagatcctgagatgggcggaaagccccagcggagaaagaatcctcaagagggcctgtataatgagctgcagaaagacaagatggccgaggcctacagcgagatcggaatgaagggcgagcgcagaagaggcaagggacacgatggactgtaccagggcctgagcaccgccaccaaggatacctatgatgccctgcacatgcaggccctgcctccaaga

SEQ ID NO: 39 - RNA, 20 nt, synthetic construct
  source 1..20: mol_type = other RNA
agagtctctcagctggtaca

SEQ ID NO: 40 - RNA, 20 nt, synthetic construct
  source 1..20: mol_type = other RNA
gagtagcgcgagcacagcta

SEQ ID NO: 41 - RNA, 20 nt, synthetic construct
  source 1..20: mol_type = other RNA
tgaacaggaaataacctatg

SEQ ID NO: 42 - RNA, 20 nt, synthetic construct
  source 1..20: mol_type = other RNA
gcgctttcccgagaccgtcc

SEQ ID NO: 43 - protein, 5 aa, synthetic construct
SFAMS

SEQ ID NO: 44 - protein, 17 aa, synthetic construct
AISGSGGGTYYADSVKG

SEQ ID NO: 45 - protein, 13 aa, synthetic construct
DKILWFGEPVFDY

SEQ ID NO: 46 - protein, 11 aa, synthetic construct
RASQSVSSYLA

SEQ ID NO: 47 - protein, 7 aa, synthetic construct
DASNRAT

SEQ ID NO: 48 - protein, 9 aa, synthetic construct
QQRSNWPPT

SEQ ID NO: 49 - protein, 122 aa, synthetic construct [sequence omitted]

SEQ ID NO: 50 - protein, 107 aa, synthetic construct [sequence omitted]

SEQ ID NO: 51 - protein, 5 aa, synthetic construct
SYYMN

SEQ ID NO: 52 - protein, 17 aa, synthetic construct
GISGDPSNTYYADSVKG

SEQ ID NO: 53 - protein, 11 aa, synthetic construct
DLPLVYTGFAY

SEQ ID NO: 54 - protein, 11 aa, synthetic construct
SGDNLRHYYVY

SEQ ID NO: 55 - protein, 7 aa, synthetic construct
GDSKRPS

SEQ ID NO: 56 - protein, 10 aa, synthetic construct
QTYTGGASLV

SEQ ID NO: 57 - protein, 120 aa, synthetic construct
QVQLVESGGGLVQPGGSLRLSCAASGFTFSSYYMNWVRQAPGKGLEWVSGISGDPSNTYYADSVKGRFTISRDNSKNTLYLQMNSLRAEDTAVYYCARDLPLVYTGFAYWGQGTLVTVSS

SEQ ID NO: 58 - protein, 109 aa, synthetic construct
DIELTQPPSVSVAPGQTARISCSGDNLRHYYVYWYQQKPGQAPVLVIYGDSKRPSGIPERFSGSNSGNTATLTISGTQAEDEADYYCQTYTGGASLVFGGGTKLTVLGQ

SEQ ID NO: 59 - protein, 5 aa, synthetic construct
DYWMQ

SEQ ID NO: 60 - protein, 17 aa, synthetic construct
TIYPGDGDTGYAQKFQG

SEQ ID NO: 61 - protein, 11 aa, synthetic construct
GDYYGSNSLDY

SEQ ID NO: 62 - protein, 11 aa, synthetic construct
KASQDVSTVVA

SEQ ID NO: 63 - protein, 7 aa, synthetic construct
SASYRYI

SEQ ID NO: 64 - protein, 9 aa, synthetic construct
QQHYSPPYT

SEQ ID NO: 65 - protein, 120 aa, synthetic construct [sequence omitted]

SEQ ID NO: 66 - protein, 107 aa, synthetic construct [sequence omitted]

SEQ ID NO: 67 - protein, 5 aa, synthetic construct
SYAIS

SEQ ID NO: 68 - protein, 17 aa, synthetic construct
RIIRFLGIANYAQKFQG

SEQ ID NO: 69 - protein, 12 aa, synthetic construct
EPGERDPDAVDI

SEQ ID NO: 70 - protein, 11 aa, synthetic construct
RASQGISNYLA

SEQ ID NO: 71 - protein, 7 aa, synthetic construct
AASSLQS

SEQ ID NO: 72 - protein, 9 aa, synthetic construct
QQYNSYPYT

SEQ ID NO: 73 - protein, 121 aa, synthetic construct
QVQLVQSGAEVKKPGSSVKVSCKAFGGTFSSYAISWVRQAPGQGLEWMGRIIRFLGIANYAQKFQGRVTLIADKSTNTAYMELSSLRSEDTAVYYCAGEPGERDPDAVDIWGQGTMVTVSS

SEQ ID NO: 74 - protein, 107 aa, synthetic construct
DIQMTQSPSSLSASVGDRVTITCRASQGISNYLAWFQQKPGKAPKSLIYAASSLQSGVPSRFSGSGSGTDFTLTISSLQPEDFATYYCQQYNSYPYTFGQGTKLEIK

SEQ ID NO: 75 - DNA, 66 bp, synthetic construct
  source 1..66: mol_type = other DNA
gtgaaacagactttgaattttgaccttctgaagttggcaggagacgttgagtccaaccctgggccc

SEQ ID NO: 76 - DNA, 432 bp, synthetic construct
  source 1..432: mol_type = other DNA
atctggagcgccgtgttcctgaacagcctgttcaaccaggaggtgcagatccccctgaccgagagctactgcggcccctgccccaagaactggatctgctacaagaacaactgctaccagttcttcgacgagagcaagaactggtacgagagccaggccagctgcatgagccagaacgccagcctgctgaaggtgtacagcaaggaggaccaggacctgctgaagctggtgaagagctaccactggatgggcctggtgcacatccccaccaacggcagctggcagtgggaggacggcagcatcctgagccccaacctgctgaccatcatcgagatgcagaagggcgactgcgccctgtacgccagcagcttcaagggctacatcgagaactgcagcacccccaacacctacatctgcatgcagcggaccgtg

SEQ ID NO: 77 - protein, 215 aa, synthetic construct
GWIRGRRSRHSWEMSEFHNYNLDLKKSDFSTRWQKQRCPVVKSKCRENASPFFFCCFIAVAMGIRFIIMVAIWSAVFLNSLFNQEVQIPLTESYCGPCPKNWICYKNNCYQFFDESKNWYESQASCMSQNASLLKVYSKEDQDLLKLVKSYHWMGLVHIPTNGSWQWEDGSILSPNLLTIIEMQKGDCALYASSFKGYIENCSTPNTYICMQRTV

SEQ ID NO: 78 - DNA, 987 bp, synthetic construct
  source 1..987: mol_type = other DNA
atgagagtgaagttcagcaggagcgcagacgcccccgcgtaccagcagggccagaaccagctctataacgagctcaatctaggacgaagagaggagtacgatgttttggacaagagacgtggccgggaccctgagatggggggaaagccgcagagaaggaagaaccctcaggaaggcctgtacaatgaactgcagaaagataagatggcggaggcctacagtgagattgggatgaaaggcgagcgccggaggggcaaggggcacgatggcctttaccagggtctcagtacagccaccaaggacacctacgacgcccttcacatgcaggccctgccccctcgcgggtggattcgtggtcggaggtctcgacacagctgggagatgagtgaatttcataattataacttggatctgaagaagagtgatttttcaacacgatggcaaaagcaaagatgtccagtagtcaaaagcaaatgtagagaaaatgcatctccattttttttctgctgcttcatcgctgtagccatgggaatccgtttcattattatggtagctatatggagtgctgtattcctaaactcattattcaaccaagaagttcaaattcccttgaccgaaagttactgtggcccatgtcctaaaaactggatatgttacaaaaataactgctaccaattttttgatgagagtaaaaactggtatgagagccaggcttcttgtatgtctcaaaatgccagccttctgaaagtatacagcaaagaggaccaggatttacttaaactggtgaagtcatatcattggatgggactagtacacattccaacaaatggatcttggcagtgggaagatggctccattctctcacccaacctactaacaataattgaaatgcagaagggagactgtgcactctatgcctcgagctttaaaggctatatagaaaactgttcaactccaaatacatacatctgcatgcaaaggactgtg

SEQ ID NO: 79 - DNA, 1167 bp, synthetic construct
  source 1..1167: mol_type = other DNA
atggcgctccctgtcaccgccttgctcctgccgctggccttgctgctccacgccgccaggccgatatggagtgctgtattcctaaactcattattcaaccaagaagttcaaattcccttgaccgaaagttactgtggcccatgtcctaaaaactggatatgttacaaaaataactgctaccaattttttgatgagagtaaaaactggtatgagagccaggcttcttgtatgtctcaaaatgccagccttctgaaagtatacagcaaagaggaccaggatttacttaaactggtgaagtcatatcattggatgggactagtacacattccaacaaatggatcttggcagtgggaagatggctccattctctcacccaacctactaacaataattgaaatgcagaagggagactgtgcactctatgcctcgagctttaaaggctatatagaaaactgttcaactccaaatacatacatctgcatgcaaaggactgtgaccacgacgccagcgccgcgaccaccaacaccggcgcccaccatcgcgtcgcagcccctgtccctgcgcccagaggcgtgccggccagcggcggggggcgcagtgcacacgagggggctggacttcgcctgtgatatctacatctgggcgcccttggccgggacttgtggggtccttctcctgtcactggttatcaccctttactgcaaacggggcagaaagaaactcctgtatatattcaaacaaccatttatgagaccagtacaaactactcaagaggaagatggctgtagctgccgatttccagaagaagaagaaggaggatgtgaactgagagtgaagttcagcaggagcgcagacgcccccgcgtaccagcagggccagaaccagctctataacgagctcaatctaggacgaagagaggagtacgatgttttggacaagagacgtggccgggaccctgagatggggggaaagccgcagagaaggaagaaccctcaggaaggcctgtacaatgaactgcagaaagataagatggcggaggcctacagtgagattgggatgaaaggcgagcgccggaggggcaaggggcacgatggcctttaccagggtctcagtacagccaccaaggacacctacgacgcccttcacatgcaggccctgccccctcgc

SEQ ID NO: 80 - DNA, 873 bp, synthetic construct
  source 1..873: mol_type = other DNA
atgaccaaggagtatcaagaccttcagcatctggacaatgaggagagtgaccaccatcagctcagaaaagggccacctcctccccagcccctcctgcagcgtctctgctccggacctcgcctcctcctgctctccctgggcctcagcctcctgctgcttgtggttgtctgtgtgatcggatcccaaaactcccagctgcaggaggagctgcggggcctgagagagacgttcagcaacttcacagcgagcacggaggcccaggtcaagggcttgagcacccagggaggcaatgtgggaagaaagatgaagtcgctagagtcccagctggagaaacagcagaaggacctgagtgaagatcactccagcctgctgctccacgtgaagcagttcgtgtctgacctgcggagcctgagctgtcagatggcggcgctccagggcaatggctcagaaaggacctgctgcccggtcaactgggtggagcacgagcgcagctgctactggttctctcgctccgggaaggcctgggctgacgccgacaactactgccggctggaggacgcgcacctggtggtggtcacgtcctgggaggagcagaaatttgtccagcaccacataggccctgtgaacacctggatgggcctccacgaccaaaacgggccctggaagtgggtggacgggacggactacgagacgggcttcaagaactggaggccggagcagccggacgactggtacggccacgggctcggaggaggcgaggactgtgcccacttcaccgacgacggccgctggaacgacgacgtctgccagaggccctaccgctgggtctgcgagacagagctggacaaggccagccaggagccacctctcctt

SEQ ID NO: 81 - DNA, 762 bp, synthetic construct
  source 1..762: mol_type = other DNA
atggaatacgcctctgacgcttcactggaccccgaagccccgtggcctcccgcgccccgcgctcgcgcctgccgcgtactgccttgggccctggtcgcggggctgctgctgctgctgctgctcgctgccgcctgcgccgtcttcctcgcctgcccctgggccgtgtccggggctcgcgcctcgcccggctccgcggccagcccgagactccgcgagggtcccgagctttcgcccgacgatcccgccggcctcttggacctgcggcagggcatgtttgcgcagctggtggcccaaaatgttctgctgatcgatgggcccctgagctggtacagtgacccaggcctggcaggcgtgtccctgacggggggcctgagctacaaagaggacacgaaggagctggtggtggccaaggctggagtctactatgtcttctttcaactagagctgcggcgcgtggtggccggcgagggctcaggctccgtttcacttgcgctgcacctgcagccactgcgctctgctgctggggccgccgccctggctttgaccgtggacctgccacccgcctcctccgaggctcggaactcggccttcggtttccagggccgcttgctgcacctgagtgccggccagcgcctgggcgtccatcttcacactgaggccagggcacgccatgcctggcagcttacccagggcgccacagtcttgggactcttccgggtgacccccgaaatcccagccggactcccttcaccgaggtcggaa

SEQ ID NO: 82 - DNA, 1698 bp, synthetic construct
  source 1..1698: mol_type = other DNA
atggccttaccagtgaccgccttgctcctgccgctggccttgctgctccacgccgccaggccggaggtgcaattgctggagtctgggggaggcttggtacagcctggggggtccctgagactctcctgtgcagcctccggattcacctttagcagttatgccatgagctgggtccgccaggctccagggaaggggctggagtgggtctcagctattagtggtagtggtggtagcacatactacgcagactccgtgaagggccggttcaccatctccagagacaattccaagaacacgctgtatctgcagatgaacagcctgagagccgaggacacggccgtatattactgtgcgaaagatgattctttctacggtggtttcgactactggggccaaggaaccctggtcaccgtctcgagtggtggaggcggttcaggcggaggtggttctggcggtggcggatcggacatccagatgacccagtctccttccaccctgtctgcatctgtaggagaccgtgtcaccatcacttgccgtgccagtcagagtattagtagctggttggcctggtatcagcagaaaccagggaaagcccctaagctcctgatctatgatgcctccagtttggaaagtggggtcccatcacgtttcagcggcagtggatccgggacagaattcactctcaccatcagcagcttgcagcctgatgattttgcaacttattactgccaacagtactcttcttacaaatacacgtttggccagggcaccaaagtcgagatcaagcgtggacaagatgcaagttctgctggatcaaccaggaataaagatccaacaagacgtccagaactagaagctggtacaaatggaagaagttcgacaacaagtccctttgtaaaaccaaatccaggttctagcacagacggcaacagcgccggacattcggggaacaacatcctcggttccgaagtggccttatttgcactcatgtacgtggcagcggccgccttcgtgctcctgttctttgtgggctgtggggtgctgctgtcccgcaagcgccggcggatgaagctgctgagcagcatcgagcaggcctgtgacatctgccggctgaagaaactgaagtgcagcaaagaaaagcccaagtgcgccaagtgcctgaagaacaactgggagtgccggtacagccccaagaccaagagaagccccctgaccagagcccacctgaccgaggtggaaagccggctggaaagactggaacagctgtttctgctgatcttcccacgcgaggacctggacatgatcctgaagatggacagcctgcaggacatcaaggccctgctgaccggcctgttcgtgcaggacaacgtgaacaaggacgccgtgaccgacagactggccagcgtggaaaccgacatgcccctgaccctgcggcagcacagaatcagcgccaccagcagcagcgaggaaagcagcaacaagggccagcggcagctgacagtgtctgctgctgcaggcggaagcggaggctctggcggatctgatgccctggacgacttcgacctggatatgctgggcagcgacgccctggatgattttgatctggacatgctgggatctgacgctctggacgatttcgatctcgacatgttgggatcagatgcactggatgactttgacctggacatgctcggatca

SEQ ID NO: 83 - protein, 494 aa, synthetic construct
MALPVTALLLPLALLLHAARPQVQLVQSGAEVKKPGASVKVSCKASGYTFTSYWMNWVRQAPGQGLEWMGRIDPYDSETHYAQKLQGRVTMTTDTSTSTAYMELRSLRSDDTAVYYCARGGYDFDVGTLYWFFDVWGQGTTVTVSSGGGGSGGGGSGGGGSDIQMTQSPSSLSASVGDRVTITCRASENIYSYLAWYQQKPGKAPKLLIYNAKTLAEGVPSRFSGSGSGTDFTLTISSLQPEDFATYYCQHHYGTPRTFGGGTKVEIKTTTPAPRPPTPAPTIASQPLSLRPEACRPAAGGAVHTRGLDFACDFWVLVVVGGVLACYSLLVTVAFIIFWVRSKRSRLLHSDYMNMTPRRPGPTRKHYQPYAPPRDFAAYRSRVKFSRSADAPAYQQGQNQLYNELNLGRREEYDVLDKRRGRDPEMGGKPQRRKNPQEGLYNELQKDKMAEAYSEIGMKGERRRGKGHDGLYQGLSTATKDTYDALHMQALPPR

SEQ ID NO: 84 - protein, 730 aa, synthetic construct
MALPVTALLLPLALLLHAARPEIVLTQSPGTLSLSPGERATLSCRASQSVSSSYLAWYQQKPGQAPRLLIYGASSRATGIPDRFSGSGSGTDFTLTISRLEPEDFAVYYCQQYKSHPITFGQGTKVEIKRGGGGSQVQLVQSGAEVKKPGASVKVSCKASGYTFTSYWMNWVRQAPGQGLEWMGRIDPYDSETHYAQKLQGRVTMTTDTSTSTAYMELRSLRSDDTAVYYCARGGYDFDVGTLYWFFDVWGQGTTVTVSSGGGGSGGGGSGGGGSDIQMTQSPSSLSASVGDRVTITCRASENIYSYLAWYQQKPGKAPKLLIYNAKTLAEGVPSRFSGSGSGTDFTLTISSLQPEDFATYYCQHHYGTPRTFGGGTKVEIKGGGGSEVQLLESGGGLVQPGGSLRLSCAASGFTFSSYAMSWVRQAPGKGLEWVSAISGSGGSTYYADSVKGRFTISRDNSKNTLYLQMNSLRAEDTAVYYCARGWPSPVTFDYWGQGTLVTVSSTTTPAPRPPTPAPTIASQPLSLRPEACRPAAGGAVHTRGLDFACDIYIWAPLAGTCGVLLLSLVITLYCKRGRKKLLYIFKQPFMRPVQTTQEEDGCSCRFPEEEEGGCELRVKFSRSADAPAYQQGQNQLYNELNLGRREEYDVLDKRRGRDPEMGGKPQRRKNPQEGLYNELQKDKMAEAYSEIGMKGERRRGKGHDGLYQGLSTATKDTYDALHMQALPPR

SEQ ID NO: 85 - protein, 731 aa, synthetic construct
MALPVTALLLPLALLLHAARPEIVLTQSPGTLSLSPGERATLSCRASQSVSSSYLAWYQQKPGQAPRLLIYGASSRATGIPDRFSGSGSGTDFTLTISRLEPEDFAVYYCQQYFNPPEYTFGQGTKVEIKRGGGGSQVQLVQSGAEVKKPGASVKVSCKASGYTFTSYWMNWVRQAPGQGLEWMGRIDPYDSETHYAQKLQGRVTMTTDTSTSTAYMELRSLRSDDTAVYYCARGGYDFDVGTLYWFFDVWGQGTTVTVSSGGGGSGGGGSGGGGSDIQMTQSPSSLSASVGDRVTITCRASENIYSYLAWYQQKPGKAPKLLIYNAKTLAEGVPSRFSGSGSGTDFTLTISSLQPEDFATYYCQHHYGTPRTFGGGTKVEIKGGGGSEVQLLESGGGLVQPGGSLRLSCAASGFTFGGNAMSWVRQAPGKGLEWVSAISGNGGSTFYADSVKGRFTISRDNSKNTLYLQMNSLRAEDTAVYYCAKVRPFWGTFDYWGQGTLVTVSSTTTPAPRPPTPAPTIASQPLSLRPEACRPAAGGAVHTRGLDFACDIYIWAPLAGTCGVLLLSLVITLYCKRGRKKLLYIFKQPFMRPVQTTQEEDGCSCRFPEEEEGGCELRVKFSRSADAPAYQQGQNQLYNELNLGRREEYDVLDKRRGRDPEMGGKPQRRKNPQEGLYNELQKDKMAEAYSEIGMKGERRRGKGHDGLYQGLSTATKDTYDALHMQALPPR

SEQ ID NO: 86 - protein, 491 aa, synthetic construct
MALPVTALLLPLALLLHAARPEVQLLESGGGLVQPGGSMRLSCAASGFTFSSYAMSWVRQAPGKGLEWVSAISGSGGSTYYADSVKGRFTISRDNSKNTLYLQMNSLRAEDTAVYYCAKYEGRYVLGAMDYWGQGTLVTVSSGGGGSGGGGSGGGGSDIQMTQSPSTLSASVGDRVTITCRASQSISSWLAWYQQKPGKAPKLLIYDASSLESGVPSRFSGSGSGTEFTLTISSLQPDDFATYYCQQYFSYPLTFGQGTKVEIKRTTTPAPRPPTPAPTIASQPLSLRPEACRPAAGGAVHTRGLDFACDFWVLVVVGGVLACYSLLVTVAFIIFWVRSKRSRLLHSDYMNMTPRRPGPTRKHYQPYAPPRDFAAYRSRVKFSRSADAPAYQQGQNQLYNELNLGRREEYDVLDKRRGRDPEMGGKPQRRKNPQEGLYNELQKDKMAEAYSEIGMKGERRRGKGHDGLYQGLSTATKDTYDALHMQALPPR

SEQ ID NO: 87 - protein, 19 aa, synthetic construct
ATNFSLLKQAGDVEENPGP

SEQ ID NO: 88 - DNA, 288 bp, synthetic construct
  source 1..288: mol_type = other DNA
aagcttgatatcgaattcggagcactgtcctccgaacgtcggagcactgtcctccgaacgtcggagcactgtcctccgaacgtcggagcactgtcctccgaacggagcatgtcctccgaacgtcggagcactgtcctccgaacgactagttaggcgtgtacggtgggaggcctatataagcagagctcgtttagtgaaccgtcagatcgcctggagacgccatccacgctgttttgacctccatagaagacaccgggaccgatccagcctctcgacattcgttggatc

SEQ ID NO: 89 - DNA, 225 bp, synthetic construct
  source 1..225: mol_type = other DNA
gggcagagcgcacatcgcccacagtccccgagaagttggggggaggggtcggcaattgaaccggtgcctagagaaggtggcgcggggtaaactgggaaagtgatgtcgtgtactggctccgcctttttcccgagggtgggggagaaccgtatataagtgcagtagtcgccgtgaacgttctttttcgcaacgggtttgccgccagaacacaggtgtcgtgacgcg

SEQ ID NO: 90 - DNA, 2997 bp, synthetic construct
  source 1..2997: mol_type = other DNA
atggccttaccagtgaccgccttgctcctgccgctggccttgctgctccacgccgccaggccggaggtgcaattgctggagtctgggggaggcttggtacagcctggggggtccctgagactctcctgtgcagcctccggattcacctttggcggtaatgccatgtcctgggtccgccaggctccagggaaggggctggagtgggtctcagcaattagtggtaatggtggtagtacattctacgcagactccgtgaagggccggttcaccatctccagagacaattccaagaacacgctgtatctgcagatgaacagcctgagagccgaggacacggccgtatattactgtgcgaaagttcgtccattctggggtactttcgactactggggccaaggaaccctggtcaccgtctcgagtggtggaggcggttcaggcggaggtggttctggcggtggcggatcggaaatcgtgttaacgcagtctccaggcaccctgtctttgtctccaggggaaagagccaccctctcttgcagggccagtcagagtgttagcagcagctacttagcctggtaccagcagaaacctggccaggctcccaggctcctcatctatggagcatccagcagggccactggcatcccagacaggttcagtggcagtggatccgggacagacttcactctcaccatcagcagactggagcctgaagattttgcagtgtattactgtcagcagtacttcaacccaccagaatacacgttcggccaggggaccaaagtggaaatcaaacgtaccacgacgccagcgccgcgaccaccaacaccggcgcccaccatcgcgtcgcagcccctgtccctgcgcccagaggcgtgccggccagcggcggggggcgcagtgcacacgagggggctggacttcgcctgtgatatctacatctgggcgcccttggccgggacttgtggggtccttctcctgtcactggttatcaccctttactgcaaacggggcagaaagaaactcctgtatatattcaaacaaccatttatgagaccagtacaaactactcaagaggaagatggctgtagctgccgatttccagaagaagaagaaggaggatgtgaactgagagtgaagttcagcaggagcgcagacgcccccgcgtaccagcagggccagaaccagctctataacgagctcaatctaggacgaagagaggagtacgatgttttggacaagagacgtggccgggaccctgagatggggggaaagccgcagagaaggaagaaccctcaggaaggcctgtacaatgaactgcagaaagataagatggcggaggcctacagtgagattgggatgaaaggcgagcgccggaggggcaaggggcacgatggcctttaccagggtctcagtacagccaccaaggacacctacgacgcccttcacatgcaggccctgccccctcgcggaagcggagctactaacttcagcctgctgaagcaggctggagacgtggaggagaaccctggacctatggccttaccagtgaccgccttgctcctgccgctggccttgctgctccacgccgccaggccggaggtgcaattgctggagtctgggggaggcttggtacagcctggggggtccctgagactctcctgtgcagcctccggattcacctttagcagttatgccatgagctgggtccgccaggctccagggaaggggctggagtgggtctcagctattagtggtagtggtggtagcacatactacgcagactccgtgaagggccggttcaccatctccagagacaattccaagaacacgctgtatctgcagatgaacagcctgagagccgaggacacggccgtatattactgtgcgcgtggttggccatctccagttactttcgactactggggccaaggaaccctggtcaccgtctcgagtggtggaggcggttcaggcggaggtggttctggcggtggcggatcggaaatcgtgttaacgcagtctccaggcaccctgtctttgtctccaggggaaagagccaccctctcttgcagggccagtcagagtgttagcagcagctacttagcctggtaccagcagaaacctggccaggctcccaggctcctcatctatggagcatccagcagggccactggcatcccagacaggttcagtggcagtggatccgggacagacttcactctcaccatcagcagactggagcctgaagattttgcagtgtattactgtcagcagtacaaatctcatccaatcacgttcggccaggggaccaaagtggaaatcaaacgtaccacgacgccagcgccgcgaccaccaacaccggcgcccaccatcgcgtcgcagcccctgtccctgcgcccagaggcgtgccggccagcggcggggggcgcagtgcacacgagggggctggacttcgcctgtgatatctacatctgggcgcccttggccgggacttgtggggtccttctcctgtcactggttatcaccctttactgcaaacggggcagaaagaaactcctgtatatattcaaacaaccatttatgagaccagtacaaactactcaagaggaagatggctgtagctgccgatttccagaagaagaagaaggaggatgtgaactgagagtgaagttcagcaggagcgcagacgcccccgcgtaccagcagggccagaaccagctctataacgagctcaatctaggacgaagagaggagtacgatgttttggacaagagacgtggccgggaccctgagatggggggaaagccgcagagaaggaagaaccctcaggaaggcctgtacaatgaactgcagaaagataagatggcggaggcctacagtgagattgggatgaaaggcgagcgccggaggggcaaggggcacgatggcctttaccagggtctcagtacagccaccaaggacacctacgacgcccttcacatgcaggccctgccccctcgc

SEQ ID NO: 91 - DNA, 2997 bp, synthetic construct
  source 1..2997: mol_type = other DNA
atggctctgcctgtgacagctctgctgctgcctctggctctgcttctgcatgccgctagacctgaagtgcagctgctggaatctggcggaggactggttcaacctggcggctctctgagactgtcttgtgccgccagcggcttcacctttggcggcaatgccatgagctgggtccgacaggctcctggcaaaggccttgaatgggtgtccgccatctctggcaatggcggcagcaccttttacgccgactctgtgaagggcagattcaccatcagccgggacaacagcaagaacaccctgtatctgcagatgaacagcctgagagccgaggacaccgccgtgtactactgtgctaaagtgcggcctttctggggcaccttcgattattggggccagggcacactggtcacagtgtctagcggaggcggaggttctggcggcggaggaagtggtggcggaggctctgaaattgtgctgacacagagccccggcacactgtctcttagccctggcgaaagagccacactgagctgtagagccagccagagcgtgtccagctcttacctggcttggtatcagcagaagcccggacaggcacccagactgctgatctatggcgcctcctctagagctacaggcatccccgatagattttccggcagcggctctggcaccgacttcaccctgacaatcagcagactggaacccgaggactttgccgtgtattattgccagcagtacttcaaccctcctgagtacaccttcggacagggcaccaaggtggaaatcaagcgcaccacaacacccgctcctagacctccaacaccagctccaacaatcgccagccagcctctgtctctgaggccagaagcttgtagacctgctgctggcggagccgtgcatacaagaggactggatttcgcctgcgacatctacatctgggcccctctggctggaacatgtggcgttctgctgctgagcctggtcatcaccctgtactgcaagcggggcagaaagaagctgctgtacatcttcaagcagcccttcatgcggcccgtgcagaccacacaagaggaagatggctgctcctgcagattccccgaggaagaagaaggcggctgcgagctgagagtgaagttcagcagatccgccgacgctcctgcctatcagcagggacagaaccagctgtacaacgagctgaacctcgggagaagagaagagtacgacgtgctggacaagcggagaggcagagatcctgagatgggcggaaagccccagcggagaaagaatcctcaagagggcctgtataatgagctgcagaaagacaagatggccgaggcctacagcgagatcggaatgaagggcgagcgcagaagaggcaagggacacgatggactgtaccagggcctgagcaccgccaccaaggatacctatgatgccctgcacatgcaggccctgcctccaagaggaagcggagctactaacttcagcctgctgaagcaggctggagacgtggaggagaaccctgggcccatggcactgccagttactgccctgctgctcccacttgcactgctgcttcatgctgccagacctgaggtccagctgttggaaagtggcggtggtcttgtgcagcctggcggaagcctcagacttagctgtgccgcctccggcttcacattcagcagctacgccatgtcctgggttcgacaagcacccggaaaaggattggagtgggtttcagccatcagcggcagcggaggcagcacttattatgccgatagcgtgaaaggccggttcaccatctccagagacaactccaagaatacgctctatctccagatgaactctctgcgcgccgaagatacagctgtgtactattgcgccagaggctggccctctcctgtgacctttgattactggggacaagggaccctcgtgaccgtttcttctggtggcggcggtagtggcggaggtggaagtggcggtggtggaagcgaaatcgtgctgacccagtctcctggaactctgtctctgtcccctggcgagagggctaccctgtcttgtagagcctctcagtccgtgtcctccagctatctcgcctggtatcaacaaaagcctgggcaagcccctcggctgctgatatacggggcttcttctcgcgccaccggcattccagacagattcagcggatctggaagcggcacagatttcacactgaccatctctcggctggaacctgaagatttcgctgtctactactgtcagcagtacaagtctcaccccatcacctttggccagggaacaaaggtcgagatcaagagaaccaccacaccagcacctaggccacctactccagctcctaccattgcctctcaacccctgagcctcagacctgaggcatgtagaccagccgcaggcggcgctgttcacacaagaggcctcgactttgcctgtgatatctatatttgggctcccctggccgggacctgcggagttcttctgctgtctctcgtgatcacactgtattgcaagagaggccggaagaagctcctctatatctttaaacagccgtttatgcgcccggtccagactacccaagaagaggacggctgtagctgtcggttccctgaagaggaagaaggcggttgcgaactgcgcgtgaaattctccagaagcgctgacgcccctgcttatcagcaaggccagaatcagctctataacgaactcaatctcggcaggcgcgaggaatatgatgtgctggataagaggcgcggcagggacccagaaatgggaggaaaacctcagcggcggaaaaacccacaagaaggcctttacaacgaactgcaaaaggataagatggcagaagcttactccgagattggcatgaagggcgaacgtcggagaggaaaaggccacgacggactctatcagggactgtctacagccacaaaggacacatacgacgcactccatatgcaggctctcccacctaga

SEQ ID NO: 92 - DNA, 2997 bp, synthetic construct
  source 1..2997: mol_type = other DNA
atggccttaccagtgaccgccttgctcctgccgctggccttgctgctccacgccgccaggccggaggtgcaattgctggagtctgggggaggcttggtacagcctggggggtccctgagactctcctgtgcagcctccggattcacctttagcagttatgccatgagctgggtccgccaggctccagggaaggggctggagtgggtctcagctattagtggtagtggtggtagcacatactacgcagactccgtgaagggccggttcaccatctccagagacaattccaagaacacgctgtatctgcagatgaacagcctgagagccgaggacacggccgtatattactgtgcgcgtggttggccatctccagttactttcgactactggggccaaggaaccctggtcaccgtctcgagtggtggaggcggttcaggcggaggtggttctggcggtggcggatcggaaatcgtgttaacgcagtctccaggcaccctgtctttgtctccaggggaaagagccaccctctcttgcagggccagtcagagtgttagcagcagctacttagcctggtaccagcagaaacctggccaggctcccaggctcctcatctatggagcatccagcagggccactggcatcccagacaggttcagtggcagtggatccgggacagacttcactctcaccatcagcagactggagcctgaagattttgcagtgtattactgtcagcagtacaaatctcatccaatcacgttcggccaggggaccaaagtggaaatcaaacgtaccacgacgccagcgccgcgaccaccaacaccggcgcccaccatcgcgtcgcagcccctgtccctgcgcccagaggcgtgccggccagcggcggggggcgcagtgcacacgagggggctggacttcgcctgtgatatctacatctgggcgcccttggccgggacttgtggggtccttctcctgtcactggttatcaccctttactgcaaacggggcagaaagaaactcctgtatatattcaaacaaccatttatgagaccagtacaaactactcaagaggaagatggctgtagctgccgatttccagaagaagaagaaggaggatgtgaactgagagtgaagttcagcaggagcgcagacgcccccgcgtaccagcagggccagaaccagctctataacgagctcaatctaggacgaagagaggagtacgatgttttggacaagagacgtggccgggaccctgagatggggggaaagccgcagagaaggaagaaccctcaggaaggcctgtacaatgaactgcagaaagataagatggcggaggcctacagtgagattgggatgaaaggcgagcgccggaggggcaaggggcacgatggcctttaccagggtctcagtacagccaccaaggacacctacgacgcccttcacatgcaggccctgccccctcgcggaagcggagctactaacttcagcctgctgaagcaggctggagacgtggaggagaaccctggacctatggccttaccagtgaccgccttgctcctgccgctggccttgctgctccacgccgccaggccggaggtgcaattgctggagtctgggggaggcttggtacagcctggggggtccctgagactctcctgtgcagcctccggattcacctttggcggtaatgccatgtcctgggtccgccaggctccagggaaggggctggagtgggtctcagcaattagtggtaatggtggtagtacattctacgcagactccgtgaagggccggttcaccatctccagagacaattccaagaacacgctgtatctgcagatgaacagcctgagagccgaggacacggccgtatattactgtgcgaaagttcgtccattctggggtactttcgactactggggccaaggaaccctggtcaccgtctcgagtggtggaggcggttcaggcggaggtggttctggcggtggcggatcggaaatcgtgttaacgcagtctccaggcaccctgtctttgtctccaggggaaagagccaccctctcttgcagggccagtcagagtgttagcagcagctacttagcctggtaccagcagaaacctggccaggctcccaggctcctcatctatggagcatccagcagggccactggcatcccagacaggttcagtggcagtggatccgggacagacttcactctcaccatcagcagactggagcctgaagattttgcagtgtattactgtcagcagtacttcaacccaccagaatacacgttcggccaggggaccaaagtggaaatcaaacgtaccacgacgccagcgccgcgaccaccaacaccggcgcccaccatcgcgtcgcagcccctgtccctgcgcccagaggcgtgccggccagcggcggggggcgcagtgcacacgagggggctggacttcgcctgtgatatctacatctgggcgcccttggccgggacttgtggggtccttctcctgtcactggttatcaccctttactgcaaacggggcagaaagaaactcctgtatatattcaaacaaccatttatgagaccagtacaaactactcaagaggaagatggctgtagctgccgatttccagaagaagaagaaggaggatgtgaactgagagtgaagttcagcaggagcgcagacgcccccgcgtaccagcagggccagaaccagctctataacgagctcaatctaggacgaagagaggagtacgatgttttggacaagagacgtggccgggaccctgagatggggggaaagccgcagagaaggaagaaccctcaggaaggcctgtacaatgaactgcagaaagataagatggcggaggcctacagtgagattgggatgaaaggcgagcgccggaggggcaaggggcacgatggcctttaccagggtctcagtacagccaccaaggacacctacgacgcccttcacatgcaggccctgccccctcgc

SEQ ID NO: 93 - DNA, 2181 bp, synthetic construct
  source 1..2181: mol_type = other DNA
atggctctgcctgtgacagctctgctgctgcctctggctctgcttctgcatgccgctagacctgaaattgtgctgacacagagccccggcacactgtctcttagccctggcgaaagagccacactgagctgtagagccagccagagcgtgtccagctcttacctggcttggtatcagcagaagcccggacaggcacccagactgctgatctatggcgcctcctctagagctacaggcatccccgatagattttccggcagcggctctggcaccgacttcaccctgacaatcagcagactggaacccgaggactttgccgtgtattattgccagcagtacttcaaccctcctgagtacaccttcggacagggcaccaaggtggaaatcaagcgcggaggcggaggttctgaggtccagctgttggaaagtggcggtggtcttgtgcagcctggcggaagcctcagacttagctgtgccgcctccggcttcacattcagcagctacgccatgtcctgggttcgacaagcacccggaaaaggattggagtgggtttcagccatcagcggcagcggaggcagcacttattatgccgatagcgtgaaaggccggttcaccatctccagagacaactccaagaatacgctctatctccagatgaactctctgcgcgccgaagatacagctgtgtactattgcgccagaggctggccctctcctgtgacctttgattactggggacaagggaccctcgtgaccgtttcttctggtggcggcggtagtggcggaggtggaagtggcggtggtggaagcgaaatcgtgctgacccagtctcctggaactctgtctctgtcccctggcgagagggctaccctgtcttgtagagcctctcagtccgtgtcctccagctatctcgcctggtatcaacaaaagcctgggcaagcccctcggctgctgatatacggggcttcttctcgcgccaccggcattccagacagattcagcggatctggaagcggcacagatttcacactgaccatctctcggctggaacctgaagatttcgctgtctactactgtcagcagtacaagtctcaccccatcacctttggccagggaacaaaggtcgagatcaagagaggtggcggaggctctgaagtgcagctgctggaatctggcggaggactggttcaacctggcggctctctgagactgtcttgtgccgccagcggcttcacctttggcggcaatgccatgagctgggtccgacaggctcctggcaaaggccttgaatgggtgtccgccatctctggcaatggcggcagcaccttttacgccgactctgtgaagggcagattcaccatcagccgggacaacagcaagaacaccctgtatctgcagatgaacagcctgagagccgaggacaccgccgtgtactactgtgctaaagtgcggcctttctggggcaccttcgattattggggccagggcacactggtcacagtgtctagcaccacaacacccgctcctagacctccaacaccagctccaacaatcgccagccagcctctgtctctgaggccagaagcttgtagacctgctgctggcggagccgtgcatacaagaggactggatttcgcctgcgacatctacatctgggcccctctggctggaacatgtggcgttctgctgctgagcctggtcatcaccctgtactgcaagcggggcagaaagaagctgctgtacatcttcaagcagcccttcatgcggcccgtgcagaccacacaagaggaagatggctgctcctgcagattccccgaggaagaagaaggcggctgcgagctgagagtgaagttcagcagatccgccgacgctcctgcctatcagcagggacagaaccagctgtacaacgagctgaacctcgggagaagagaagagtacgacgtgctggacaagcggagaggcagagatcctgagatgggcggaaagccccagcggagaaagaatcctcaagagggcctgtataatgagctgcagaaagacaagatggccgaggcctacagcgagatcggaatgaagggcgagcgcagaagaggcaagggacacgatggactgtaccagggcctgagcaccgccaccaaggatacctatgatgccctgcacatgcaggccctgcctccaaga

SEQ ID NO: 94 - DNA, 2181 bp, synthetic construct
  source 1..2181: mol_type = other DNA
atggccttaccagtgaccgccttgctcctgccgctggccttgctgctccacgccgccaggccggaaatcgtgttaacgcagtctccaggcaccctgtctttgtctccaggggaaagagccaccctctcttgcagggccagtcagagtgttagcagcagctacttagcctggtaccagcagaaacctggccaggctcccaggctcctcatctatggagcatccagcagggccactggcatcccagacaggttcagtggcagtggatccgggacagacttcactctcaccatcagcagactggagcctgaagattttgcagtgtattactgtcagcagtacttcaacccaccagaatacacgttcggccaggggaccaaagtggaaatcaaacgtggtggcggaggaagcgaggtgcaattgctggagtctgggggaggcttggtacagcctggggggtccctgagactctcctgtgcagcctccggattcacctttagcagttatgccatgagctgggtccgccaggctccagggaaggggctggagtgggtctcagctattagtggtagtggtggtagcacatactacgcagactccgtgaagggccggttcaccatctccagagacaattccaagaacacgctgtatctgcagatgaacagcctgagagccgaggacacggccgtatattactgtgcgcgtggttggccatctccagttactttcgactactggggccaaggaaccctggtcaccgtctcgagtggtggaggcggttcaggcggaggtggttctggcggtggcggatcggaaatcgtgttaacgcagtctccaggcaccctgtctttgtctccaggggaaagagccaccctctcttgcagggccagtcagagtgttagcagcagctacttagcctggtaccagcagaaacctggccaggctcccaggctcctcatctatggagcatccagcagggccactggcatcccagacaggttcagtggcagtggatccgggacagacttcactctcaccatcagcagactggagcctgaagattttgcagtgtattactgtcagcagtacaaatctcatccaatcacgttcggccaggggaccaaagtggaaatcaaacgtggaggcggcggaagcgaggtgcaattgctggagtctgggggaggcttggtacagcctggggggtccctgagactctcctgtgcagcctccggattcacctttggcggtaatgccatgtcctgggtccgccaggctccagggaaggggctggagtgggtctcagcaattagtggtaatggtggtagtacattctacgcagactccgtgaagggccggttcaccatctccagagacaattccaagaacacgctgtatctgcagatgaacagcctgagagccgaggacacggccgtatattactgtgcgaaagttcgtccattctggggtactttcgactactggggccaaggaaccctggtcaccgtctcgagtaccacgacgccagcgccgcgaccaccaacaccggcgcccaccatcgcgtcgcagcccctgtccctgcgcccagaggcgtgccggccagcggcggggggcgcagtgcacacgagggggctggacttcgcctgtgatatctacatctgggcgcccttggccgggacttgtggggtccttctcctgtcactggttatcaccctttactgcaaacggggcagaaagaaactcctgtatatattcaaacaaccatttatgagaccagtacaaactactcaagaggaagatggctgtagctgccgatttccagaagaagaagaaggaggatgtgaactgagagtgaagttcagcaggagcgcagacgcccccgcgtaccagcagggccagaaccagctctataacgagctcaatctaggacgaagagaggagtacgatgttttggacaagagacgtggccgggaccctgagatggggggaaagccgcagagaaggaagaaccctcaggaaggcctgtacaatgaactgcagaaagataagatggcggaggcctacagtgagattgggatgaaaggcgagcgccggaggggcaaggggcacgatggcctttaccagggtctcagtacagccaccaaggacacctacgacgcccttcacatgcaggccctgccccctcgc

SEQ ID NO: 95 - DNA, 2181 bp, synthetic construct
  source 1..2181: mol_type = other DNA
atggctctgcctgtgacagctctgctgctgcctctggctctgcttctgcatgccgctagacctgaaatcgtgctgacccagtctcctggaactctgtctctgtcccctggcgagagggctaccctgtcttgtagagcctctcagtccgtgtcctccagctatctcgcctggtatcaacaaaagcctgggcaagcccctcggctgctgatatacggggcttcttctcgcgccaccggcattccagacagattcagcggatctggaagcggcacagatttcacactgaccatctctcggctggaacctgaagatttcgctgtctactactgtcagcagtacaagtctcaccccatcacctttggccagggaacaaaggtcgagatcaagagaggtggcggcggtagtgaagtgcagctgctggaatctggcggaggactggttcaacctggcggctctctgagactgtcttgtgccgccagcggcttcacctttggcggcaatgccatgagctgggtccgacaggctcctggcaaaggccttgaatgggtgtccgccatctctggcaatggcggcagcaccttttacgccgactctgtgaagggcagattcaccatcagccgggacaacagcaagaacaccctgtatctgcagatgaacagcctgagagccgaggacaccgccgtgtactactgtgctaaagtgcggcctttctggggcaccttcgattattggggccagggcacactggtcacagtgtctagcggaggcggaggttctggcggcggaggaagtggtggcggaggctctgaaattgtgctgacacagagccccggcacactgtctcttagccctggcgaaagagccacactgagctgtagagccagccagagcgtgtccagctcttacctggcttggtatcagcagaagcccggacaggcacccagactgctgatctatggcgcctcctctagagctacaggcatccccgatagattttccggcagcggctctggcaccgacttcaccctgacaatcagcagactggaacccgaggactttgccgtgtattattgccagcagtacttcaaccctcctgagtacaccttcggacagggcaccaaggtggaaatcaagcgcggcggtggtggaagcgaggtccagctgttggaaagtggcggtggtcttgtgcagcctggcggaagcctcagacttagctgtgccgcctccggcttcacattcagcagctacgccatgtcctgggttcgacaagcacccggaaaaggattggagtgggtttcagccatcagcggcagcggaggcagcacttattatgccgatagcgtgaaaggccggttcaccatctccagagacaactccaagaatacgctctatctccagatgaactctctgcgcgccgaagatacagctgtgtactattgcgccagaggctggccctctcctgtgacctttgattactggggacaagggaccctcgtgaccgtttcttctaccacaacacccgctcctagacctccaacaccagctccaacaatcgccagccagcctctgtctctgaggccagaagcttgtagacctgctgctggcggagccgtgcatacaagaggactggatttcgcctgcgacatctacatctgggcccctctggctggaacatgtggcgttctgctgctgagcctggtcatcaccctgtactgcaagcggggcagaaagaagctgctgtacatcttcaagcagcccttcatgcggcccgtgcagaccacacaagaggaagatggctgctcctgcagattccccgaggaagaagaaggcggctgcgagctgagagtgaagttcagcagatccgccgacgctcctgcctatcagcagggacagaaccagctgtacaacgagctgaacctcgggagaagagaagagtacgacgtgctggacaagcggagaggcagagatcctgagatgggcggaaagccccagcggagaaagaatcctcaagagggcctgtataatgagctgcagaaagacaagatggccgaggcctacagcgagatcggaatgaagggcgagcgcagaagaggcaagggacacgatggactgtaccagggcctgagcaccgccaccaaggatacctatgatgccctgcacatgcaggccctgcctccaaga

SEQ ID NO: 96 - protein, 677 aa, synthetic construct
EIVLTQSPGTLSLSPGERATLSCRASQSVSSSYLAWYQQKPGQAPRLLIYGASSRATGIPDRFSGSGSGTDFTLTISRLEPEDFAVYYCQQYFNPPEYTFGQGTKVEIKRGGGGSEVQLLESGGGLVQPGGSLRLSCAASGFTFSSYAMSWVRQAPGKGLEWVSAISGSGGSTYYADSVKGRFTISRDNSKNTLYLQMNSLRAEDTAVYYCARGWPSPVTFDYWGQGTLVTVSSGGGGSGGGGSGGGGSEIVLTQSPGTLSLSPGERATLSCRASQSVSSSYLAWYQQKPGQAPRLLIYGASSRATGIPDRFSGSGSGTDFTLTISRLEPEDFAVYYCQQYKSHPITFGQGTKVEIKRGGGGSEVQLLESGGGLVQPGGSLRLSCAASGFTFGGNAMSWVRQAPGKGLEWVSAISGNGGSTFYADSVKGRFTISRDNSKNTLYLQMNSLRAEDTAVYYCAKVRPFWGTFDYWGQGTLVTVSSESKYGPPCPPCPMFWVLVVVGGVLACYSLLVTVAFIIFWVKRGRKKLLYIFKQPFMRPVQTTQEEDGCSCRFPEEEEGGCELRVKFSRSADAPAYQQGQNQLYNELNLGRREEYDVLDKRRGRDPEMGGKPQRRKNPQEGLYNELQKDKMAEAYSEIGMKGERRRGKGHDGLYQGLSTATKDTYDALHMQALPPR

SEQ ID NO: 97 - protein, 467 aa, synthetic construct
EVQLLESGGGLVQPGGSLRLSCAASGFTFSSYAMSWVRQAPGKGLEWVSAISGSGGSTYYADSVKGRFTISRDNSKNTLYLQMNSLRAEDTAVYYCARGWPSPVTFDYWGQGTLVTVSSGGGGSGGGGSGGGGSEIVLTQSPGTLSLSPGERATLSCRASQSVSSSYLAWYQQKPGQAPRLLIYGASSRATGIPDRFSGSGSGTDFTLTISRLEPEDFAVYYCQQYKSHPITFGQGTKVEIKRTTTPAPRPPTPAPTIASQPLSLRPEACRPAAGGAVHTRGLDFACDIYIWAPLAGTCGVLLLSLVITLYCKRGRKKLLYIFKQPFMRPVQTTQEEDGCSCRFPEEEEGGCELRVKFSRSADAPAYQQGQNQLYNELNLGRREEYDVLDKRRGRDPEMGGKPQRRKNPQEGLYNELQKDKMAEAYSEIGMKGERRRGKGHDGLYQGLSTATKDTYDALHMQALPPR

SEQ ID NO: 98 - protein, 468 aa, synthetic construct
EVQLLESGGGLVQPGGSLRLSCAASGFTFGGNAMSWVRQAPGKGLEWVSAISGNGGSTFYADSVKGRFTISRDNSKNTLYLQMNSLRAEDTAVYYCAKVRPFWGTFDYWGQGTLVTVSSGGGGSGGGGSGGGGSEIVLTQSPGTLSLSPGERATLSCRASQSVSSSYLAWYQQKPGQAPRLLIYGASSRATGIPDRFSGSGSGTDFTLTISRLEPEDFAVYYCQQYFNPPEYTFGQGTKVEIKRTTTPAPRPPTPAPTIASQPLSLRPEACRPAAGGAVHTRGLDFACDIYIWAPLAGTCGVLLLSLVITLYCKRGRKKLLYIFKQPFMRPVQTTQEEDGCSCRFPEEEEGGCELRVKFSRSADAPAYQQGQNQLYNELNLGRREEYDVLDKRRGRDPEMGGKPQRRKNPQEGLYNELQKDKMAEAYSEIGMKGERRRGKGHDGLYQGLSTATKDTYDALHMQALPPR

SEQ ID NO: 99 - protein, 119 aa, synthetic construct
EVQLLESGGGLVQPGGSLRLSCAASGFTFSSYAMSWVRQAPGKGLEWVSAISGSGGSTYYADSVKGRFTISRDNSKNTLYLQMNSLRAEDTAVYYCARGWPSPVTFDYWGQGTLVTVSS

SEQ ID NO: 100 - protein, 119 aa, synthetic construct
EVQLLESGGGLVQPGGSLRLSCAASGFTFGGNAMSWVRQAPGKGLEWVSAISGNGGSTFYADSVKGRFTISRDNSKNTLYLQMNSLRAEDTAVYYCAKVRPFWGTFDYWGQGTLVTVSS

SEQ ID NO: 101 - protein, 110 aa, synthetic construct
EIVLTQSPGTLSLSPGERATLSCRASQSVSSSYLAWYQQKPGQAPRLLIYGASSRATGIPDRFSGSGSGTDFTLTISRLEPEDFAVYYCQQYFNPPEYTFGQGTKVEIKR

SEQ ID NO: 102 - protein, 109 aa, synthetic construct
EIVLTQSPGTLSLSPGERATLSCRASQSVSSSYLAWYQQKPGQAPRLLIYGASSRATGIPDRFSGSGSGTDFTLTISRLEPEDFAVYYCQQYKSHPITFGQGTKVEIKR

SEQ ID NO: 103 - protein, 243 aa, synthetic construct
EVQLLESGGGLVQPGGSLRLSCAASGFTFSSYAMSWVRQAPGKGLEWVSAISGSGGSTYYADSVKGRFTISRDNSKNTLYLQMNSLRAEDTAVYYCARGWPSPVTFDYWGQGTLVTVSSGGGGSGGGGSGGGGSEIVLTQSPGTLSLSPGERATLSCRASQSVSSSYLAWYQQKPGQAPRLLIYGASSRATGIPDRFSGSGSGTDFTLTISRLEPEDFAVYYCQQYKSHPITFGQGTKVEIKR

SEQ ID NO: 104 - protein, 5 aa, synthetic construct
SYAMS

SEQ ID NO: 105 - protein, 17 aa, synthetic construct
AISGSGGSTYYADSVKG

SEQ ID NO: 106 - protein, 10 aa, synthetic construct
GWPSPVTFDY

SEQ ID NO: 107 - protein, 12 aa, synthetic construct
RASQSVSSSYLA

SEQ ID NO: 108 - protein, 7 aa, synthetic construct
GASSRAT

SEQ ID NO: 109 - protein, 9 aa, synthetic construct
QQYKSHPIT

SEQ ID NO: 110 - protein, 5 aa, synthetic construct
GNAMS

SEQ ID NO: 111 - protein, 17 aa, synthetic construct
AISGNGGSTFYADSVKG

SEQ ID NO: 112 - protein, 10 aa, synthetic construct
VRPFWGTFDY

SEQ ID NO: 113 - protein, 12 aa, synthetic construct
RASQSVSSSYLA

SEQ ID NO: 114 - protein, 7 aa, synthetic construct
GASSRAT

SEQ ID NO: 115 - protein, 10 aa, synthetic construct
QQYFNPPEYT

SEQ ID NO: 116 - protein, 125 aa, synthetic construct
QVQLVQSGAEVKKPGASVKVSCKASGYTFTSYWMNWVRQAPGQGLEWMGRIDPYDSETHYAQKLQGRVTMTTDTSTSTAYMELRSLRSDDTAVYYCARGGYDFDVGTLYWFFDVWGQGTTVTVSS

SEQ ID NO: 117 - protein, 107 aa, synthetic construct
DIQMTQSPSSLSASVGDRVTITCRASENIYSYLAWYQQKPGKAPKLLIYNAKTLAEGVPSRFSGSGSGTDFTLTISSLQPEDFATYYCQHHYGTPRTFGGGTKVEIK